European Patent Specification EP 3 298 163 B1, published September 6, 2023. Title: DIAGNOSTIC METHOD. Applicant: NATIONAL UNIVERSITY OF IRELAND, GALWAY. The sequence listing filed with the application follows.

SEQUENCE LISTING (193 sequences)

SEQ ID NO: 1 - DNA, 486 bp, Haemophilus influenzae
atgacaaagaaaaaagtaaaacccaattcaaatactatcgcactaaataaacgtgcaagacacgattattttattgaagatgaaattgaagcaggtcttgaattacaaggctgggaagtcaaatctatgcgcgcaggcaaggcaaatattagtgatagttatgttatttttaaaaatggcgaagcctttttattcggcgcaagcattcagccattaaatgttgcatcaacgcatattgtttgtgatccaactcgcactcgtaagttattgttaaataaacgcgaattagcatccctatttggtaaagcaaaccgagacggttttaccatagttgcactttctctttattggaaaagtgcgtgggcaaaagtcaaaatcggtttagccaaaggtaaaaaacaacaggataaacgtgatgatattaaagaacgtgaatggaaagtaacaaaagatcgcattatgaaaaatgcacatcgaagatcttaa

SEQ ID NO: 2 - protein, 161 aa, Haemophilus influenzae
MTKKKVKPNSNTIALNKRARHDYFIEDEIEAGLELQGWEVKSMRAGKANISDSYVIFKNGEAFLFGASIQPLNVASTHIVCDPTRTRKLLLNKRELASLFGKANRDGFTIVALSLYWKSAWAKVKIGLAKGKKQQDKRDDIKEREWKVTKDRIMKNAHRRS

SEQ ID NO: 3 - DNA, 20 bp, Artificial Sequence
  H. influenzae smpB F1
attaaatgtygcatcaacgc

SEQ ID NO: 4 - DNA, 17 bp, Artificial Sequence
  H. influenzae smpB R1
gacttttgcccacgcac

SEQ ID NO: 5 - DNA, 27 bp, Artificial Sequence
  H. influenzae smpB P1
acgrttttaccatagttgcactttctc

SEQ ID NO: 6 - DNA, 21 bp, Artificial Sequence
  MTC FwP
caaggcacggaggtgaagagc

SEQ ID NO: 7 - DNA, 17 bp, Artificial Sequence
  Bacillus subtilis F1
aacgtagcattagctgc

SEQ ID NO: 8 - DNA, 17 bp, Artificial Sequence
  Bacillus subtilis R1
ctcatcttcttgcctgc

SEQ ID NO: 9 - DNA, 21 bp, Artificial Sequence
  Bacillus subtilis P1
cacatccaagtaggctacgct

SEQ ID NO: 10 - DNA, 22 bp, Artificial Sequence
  LegPneuF1
cacgtgataatmaaatacggtg

SEQ ID NO: 11 - DNA, 21 bp, Artificial Sequence
  MTC RvP
ctcgtggttggtccagctgcc

SEQ ID NO: 12 - DNA, 19 bp, Artificial Sequence
  LegPneuR1
ttcatcaayagcttgcgyg

SEQ ID NO: 13 - DNA, 28 bp, Artificial Sequence
  MTC_P
caggcgtcgctggccgattcgttcgcca

SEQ ID NO: 14 - DNA, 26 bp, Artificial Sequence
  LegPneuP3
cygcatccactcattttattcctgat

SEQ ID NO: 15 - DNA, 20 bp, Artificial Sequence
  A.baum smpB F1
tggcatgtctttactaggct

SEQ ID NO: 16 - DNA, 22 bp, Artificial Sequence
  A.baum smpB R1
gcacaatatgtgtagatgcaga

SEQ ID NO: 17 - DNA, 23 bp, Artificial Sequence
  A.baum smpB P
tggtgctcagattcaaccactcc

SEQ ID NO: 18 - DNA, 17 bp, Artificial Sequence
  L.gra smpB F1
cggcattgtcttgcaag

SEQ ID NO: 19 - DNA, 20 bp, Artificial Sequence
  L.gra smpB R1
gctgatatgcatgttgtgta

SEQ ID NO: 20 - DNA, 22 bp, Artificial Sequence
  L.gra smpB PHEX2
agttcactcgtgcattacgaac

SEQ ID NO: 21 - DNA, 19 bp, Artificial Sequence
  Mpneu_F1
ttagcatttcgccctatgc

SEQ ID NO: 22 - DNA, 19 bp, Artificial Sequence
  Mpneu_R1
agtccttcttgcttttggc

SEQ ID NO: 23 - DNA, 20 bp, Artificial Sequence
  Mpneu_P1
ccaccccttcaaacgggtga

SEQ ID NO: 24 - DNA, 19 bp, Artificial Sequence
  M. av_avp FwP
cgttgcaaggaaccgaggt

SEQ ID NO: 25 - DNA, 21 bp, Artificial Sequence
  M. av_avp RvP
gtcgtgattggtccagctacc

SEQ ID NO: 26 - DNA, 24 bp, Artificial Sequence
  M. av_avp P
caagcgtcgttagctgacgcgttc

SEQ ID NO: 27 - DNA, 19 bp, Artificial Sequence
  M. int FwP
gctgcaaggcaccgaggtc

SEQ ID NO: 28 - DNA, 21 bp, Artificial Sequence
  M. int RvP
gtcatgattggtccagctacc

SEQ ID NO: 29 - DNA, 24 bp, Artificial Sequence
  M. int P
caagcttcgttagctgacgccttc

SEQ ID NO: 30 - DNA, 18 bp, Artificial Sequence
  LgensmpB_F
gatcaatacgaagcaggc

SEQ ID NO: 31 - DNA, 20 bp, Artificial Sequence
  LgensmpB_R
gccattctctgtctttgatc

SEQ ID NO: 32 - DNA, 21 bp, Artificial Sequence
  Leg ssrA F1
ygcaaayrawgmaawsttygm

SEQ ID NO: 33 - DNA, 21 bp, Artificial Sequence
  Leg ssrA R1
ctctgccdtyaghtctacatg

SEQ ID NO: 34 - DNA, 25 bp, Artificial Sequence
  Leg ssrA P3
yggtaycgaatcaacggtcatarra

SEQ ID NO: 35 - DNA, 19 bp, Artificial Sequence
  SIAC F2
atgccagtcagcataagga

SEQ ID NO: 36 - DNA, 21 bp, Artificial Sequence
  SIAC R2
cagacctctggtaggatgtac

SEQ ID NO: 37 - DNA, 20 bp, Artificial Sequence
  H. influenzae smpB F1
attaaatgttgcatcaacgc

SEQ ID NO: 38 - DNA, 19 bp, Artificial Sequence
  LegPneuR1
ttcatcaatagcttgcgyg

SEQ ID NO: 39 - DNA, 25 bp, Artificial Sequence
  Leg ssrA P3
yggtatcgaatcaacggtcatarra

SEQ ID NO: 40 - DNA, 21 bp, Artificial Sequence
  Leg ssrA F1
tgcaaacgatgaaaactttgc

SEQ ID NO: 41 - DNA, 21 bp, Artificial Sequence
  Leg ssrA R1
ctctgcctttagctctacatg

SEQ ID NO: 42 - DNA, 20 bp, Artificial Sequence
  SIAC P1
tcggcactaccgacacgaac

SEQ ID NO: 43 - DNA, 500 bp, Artificial Sequence
  SIAC
acctctaagtaagtgagcggtcgtgacattatccctgattttctcactactattagtactcacggcgcaattccaccacagccttgtctcgccagaatgccagtcagcataaggaagagctcaaggcaggtcaactcgcactgtgagggtcacatgggcgttcggcactaccgacacgaacctcagttagcgtacatcctaccagaggtctgtggccccgtggtcaaaagtgcgggtttcgtatttgctgctcgtcagtactttcagaatcatgacctgcacggcaaagagacgcttattatggagctcgacatggcaataacgcgacgaatctacgtcacgacgagaatagtgtaaacgaagctgctgacggcggaagcgtcaaaggggtctgtgaattgttattcgcgaaaaacatccgtccccgtgggggatagtcaccgacgccgttttatagaagcctaggggaacaggttggtttaactagcttaagaaagtaa

SEQ ID NO: 44 - DNA, 471 bp, Legionella pneumophila
atgactaccaaaaaacaaccagattccaccatagccttgaatagaaaagctggttttgattattttattgaagatcaatacgaagcaggcctggttttggagggctgggaagtaaaaagtctgcgtgctgggaaaatcaatttgtcggattcacacgtgataatcaaatacggtgaggcattcctattgggcgcccaaatacagcctcttcccaccgcatccactcattttattcctgatccggtcaggacgcgcaagctattgatgaataaaaaagaattaaaccatctcattggaagtgttgaaaggcaaggctataccatagtccctctttctttgtattggaaaaaaaataaaattaaaataaaaattgctctggccaaaggaaaaaaagagcatgacaaaagagacacgatcaaagacagagaatggcaaagagatcgttcaagaataatgaaaaagaacacttga

SEQ ID NO: 45 - DNA, 471 bp, Legionella pneumophila
atgactaccaaaaaacaaccagattccaccatagccttgaatagaaaagctggttttgattactttattgaagatcaatacgaagcaggcctggttttggaaggctgggaagtaaaaagtctgcgtgctggaaaaatcaatttgtcggattcacacgtgataatcaaatacggtgaggcattcctattgggcgcccaaatacagccgcttcccaccgcatccactcattttattcctgatccgatcaggacgcgcaagctattgatgaataaaaaagaattaaaccatctcataggaagtgttgaaaggcaaggctataccatagtccctctttctttgtattggaaaaaaaataaaattaaaataaaaattgctctggccaaaggaaaaaaagagcatgacaaaagagacacgatcaaagacagagaatggcaaagggatcgttcaagaataatgaaaaagaacacttga

SEQ ID NO: 46 - DNA, 398 bp, Legionella pneumophila
atgactaccaaaaaacaaccagattccaccatagccttgaatagaaaagctggttttgattactttattgaagatcaatacgaagcaggcctggttttggaaggctgggaagtaaaaagtctgcgtgctggaaaaatcaatttgtcggattcacacgtgataatcaaatacggtgaggcattcctattgggcgcccaaatacagcctcttcccaccgcatccactcattttattcctgatccgatcaggacgcgcaagctattgatgaataaaaaagaattaaaccatctcataggaagtgttgaaaggcaaggctataccatagtccctctttctttgtattggaaaaaaaataaaattaaaataaaaattgctctggctaaaggaaaaaaagagca

SEQ ID NO: 47 - DNA, 471 bp, Legionella pneumophila
atgactaccaaaaaacaaccagattccaccatagctttgaatagaaaagctggttttgattactttattgaagatcaatacgaagcaggcctggttttggaaggctgggaagtaaaaagtctgcgtgctggaaaaatcaatttgtcggattcacacgtgataatcaaatacggtgaggcattcctattgggcgcccaaatacagcctcttccaaccgcatccactcattttattcctgatccggtcaggacgcgcaagctattgatgaataaaaaagaattaaaccatctcattggaagtgttgaaaggcaaggctataccatagtccctctttctttgtattggaaaaaaaataaaattaaaataaaaattgctctggccaaaggaaaaaaagagcatgacaaaagagacacgatcaaagacagagaatggcaaagagatcgttcaagaataatgaaaaagaacacttga

SEQ ID NO: 48 - DNA, 471 bp, Legionella pneumophila; identical to SEQ ID NO: 45

SEQ ID NO: 49 - DNA, 471 bp, Legionella pneumophila
atgactaccaaaaaacaaccagattccaccatagccttgaatagaaaagctggttttgattactttattgaagatcaatacgaagcaggcctggttttggaaggctgggaagtaaaaagtctgcgtgctggaaaaatcaatttgtcggattcacacgtgataatcaaatacggtgaggcattcctattgggcgcccaaatacagcctcttcccaccgcatccactcattttattcctgatccgatcaggacgcgcaagctattgatgaataaaaaagaattaaaccatctcataggaagtgttgaaaggcaaggctataccatagtccctctttctttgtattggaaaaaaaataaaattaaaataaaaattgctctggctaaaggaaaaaaagagcatgacaaaagagacacgatcaaagacagagaatggcaaagggatcgttcaagaataatgaaaaagaacacttga

SEQ ID NO: 50 - DNA, 471 bp, Legionella pneumophila
atgactaccaaaaaacaaccagattcaaccatagctttgaatagaaaagctggttttgattactttattgaagatcaatacgaagcaggcctggttttggaaggctgggaagtaaaaagtctgcgtgctggaaaaatcaatttgtcggattcacacgtgataatcaaatacggtgaggcattcctattgggcgcccaaatacagcctcttcccaccgcatccactcattttattcctgatccggtcaggacgcgcaagctattgatgaataaaaaagaattaaaccatctcataggaagtgttgaaaggcaaggctataccatagtccctctttctttgtattggaaaaaaaataaaattaaaataaaaattgctctggccaaaggaaaaaaagagcatgacaaaagagacacgatcaaagacagagaatggcaaagggatcgttcaagaataatgaaaaagaacacttga

SEQ ID NO: 51 - DNA, 471 bp, Legionella pneumophila
atgactaccaaaaaacaaccagattccaccatagccttgaatagaaaagctggttttgattactttattgaagatcaatacgaagcaggcctggttttggaaggctgggaagtaaaaagtctgcgtgctggaaaaatcaatttgtcggattcacacgtgataatcaaatacggtgaggcattcctattgggcgcccaaatacagcctcttcccaccgcatccactcattttattcctgatccgctgaggacgcgcaagctattgatgaataaaagagaattaaaccatctcataggaagtgttgaaaggcaaggctataccatagtccctctttctttgtattggaaaaaaaataaaattaaaataaaaattgctctggccaaaggaaaaaaagagcatgacaaaagagacacgatcaaagacagagaatggcaaagggatcgttcaagaataatgaaaaagaacacttga

SEQ ID NO: 52 - DNA, 471 bp, Legionella pneumophila; identical to SEQ ID NO: 49

SEQ ID NO: 53 - DNA, 471 bp, Legionella pneumophila; identical to SEQ ID NO: 49

SEQ ID NO: 54 - DNA, 361 bp, Legionella pneumophila
gatcaatacgaagcaggcctggttttggagggctgggaagtaaaaagtctgcgtgctgggaaaatcaatttgtcggattcacacgtgataatcaaatacggtgaggcattcctattgggcgcccaaatacagcctcttcccaccgcatccactcattttattcctgatccggtcaggacgcgcaagctattgatgaataaaaaagaattaaaccatctcattggaagtgttgaaaggcaaggctataccatagtccctctttctttgtattggaaaaaaaataaaattaaaataaaaattgctctggccaaaggaaaaaaagagcatgacaaaagagacacgatcaaagacagagaatggc

SEQ ID NO: 55 - DNA, 361 bp, Legionella pneumophila
gatcaatacgaagcaggcctggttttggaaggctgggaagtaaaaagtctgcgtgctggaaaaatcaatttgtcggattcacacgtgataatcaaatacggtgaggcattcctattgggcgcccaaatacagccgcttcccaccgcatccactcattttattcctgatccgatcaggacgcgcaagctattgatgaataaaaaagaattaaaccatctcataggaagtgttgaaaggcaaggctataccatagtccctctttctttgtattggaaaaaaaataaaattaaaataaaaattgctctggccaaaggaaaaaaagagcatgacaaaagagacacgatcaaagacagagaatggc

SEQ ID NO: 56 - DNA, 361 bp, Legionella pneumophila
gatcaatacgaagcaggcctggttttggaaggctgggaagtaaaaagtctgcgtgctggaaaaatcaatttgtcggattcacacgtgataatcaaatacggtgaggcattcctattgggcgcccaaatacagcctcttcccaccgcatccactcattttattcctgatccggtcaggacgcgcaagctattgatgaataaaaaagaattaaaccatctcattggaagtgttgaaaggcaaggctataccatagtccctctttctttgtattggaaaaaaaataaaattaaaataaaaattgctctggccaaaggaaaaaaagagcatgacaaaagagacacgatcaaagacagagaatggc

SEQ ID NO: 57 - DNA, 361 bp, Legionella pneumophila
gatcaatacgaagcaggcctggttttggaaggctgggaagtaaaaagtctgcgtgctggaaaaatcaatttgtcggattcacacgtgataatcaaatacggtgaggcattcctattgggcgcccaaatacagcctcttcccaccgcatccactcattttattcctgatccgatcaggacgcgcaagctattgatgaataaaaaagaattaaaccatctcataggaagtgttgaaaggcaaggctataccatagtccctctttctttgtattggaaaaaaaataaaattaaaataaaaattgctctggctaaaggaaaaaaagagcatgacaaaagagacacgatcaaagacagagaatggc

SEQ ID NO: 58 - DNA, 361 bp, Legionella pneumophila
gatcaatacgaagcaggcttggttttggaaggctgggaagtaaaaagtctgcgggcaggaaaaatcaatttgtcagatgcacacgtgataatcaaatacggtgaggcattcctgttaggagctcaaatacagcctcttcctactgcatccactcattttattcctgatccggtcaggacacgcaagctattgatgaataaaaaagaattaaaccatctcatcggaagtgttgaaagacaaggctataccatagtgcctctttctttgtattggaaaaagaataaaattaaaataaaaatcgctctggctaaaggaaaaaaagagcatgacaaaagagacacgatcaaagacagagaatggc

SEQ ID NO: 59 - DNA, 361 bp, Legionella pneumophila
gatcaatacgaagcaggcttggttttggaaggctgggaagtaaaaagtctgcgtgcaggaaaaatcaatttgtcggatgcacacgtgataataaaatacggtgaggcattcctgttaggagcccaaatacagcctcttcctactgcatccactcattttattcctgatccagtcaggacacgcaagctgttgatgaataaaaaagaattaaaccatcttatcggaagtgttgaaagacaaggctataccatagttcctctttctttgtattggaaaaagaataaaattaaaataaaaatcgcactggccaaaggaaagaaagagcatgacaaaagagacacgatcaaagacagagaatggc

SEQ ID NO: 60 - DNA, 361 bp, Legionella pneumophila
gatcaatacgaagcaggcctggttttggaaggctgggaagtaaaaagtctgcgtgctgggaaaatcaatttgtcggattcacacgtgataatcaaatacggtgaagcattcctattgggcgcccaaatacagcctcttcccaccgcatccactcattttattcctgatccggtcaggacgcgcaagctattgatgaataaaaaagaattaaaccatctcattggaagtgttgaaaggcaaggctataccatagtccctctttctttgtattggaaaaaaaataaaattaaaataaaaattgctctggccaaaggaaaaaaagagcatgacaaaagagacacgatcaaagacagagaatggc

SEQ ID NO: 61 - DNA, 361 bp, Legionella pneumophila; identical to SEQ ID NO: 57

SEQ ID NO: 62 - DNA, 361 bp, Legionella pneumophila
gatcaatacgaagcaggcctggttttggaaggctgggaagtaaaaagtctgcgtgctggaaaaatcaatttgtcggattcacacgtgataatcaaatacggtgaggcattcctattgggcgcccaaatacagcctcttcccaccgcatccactcattttattcctgatccgctgaggacgcgcaagctattgatgaataaaagagaattaaaccatctcataggaagtgttgaaaggcaaggctataccatagtccctctttctttgtattggaaaaaaaataaaattaaaataaaaattgctctggccaaaggaaaaaaagagcatgacaaaagagacacgatcaaagacagagaatggc

SEQ ID NO: 63 - DNA, 361 bp, Legionella pneumophila; identical to SEQ ID NO: 62

SEQ ID NO: 64 - DNA, 361 bp, Legionella pneumophila; identical to SEQ ID NO: 62

SEQ ID NO: 65 - DNA, 361 bp, Legionella pneumophila
gatcaatacgaagcaggcctggttttggaaggctgggaagtaaaaagtctgcgtgctggaaaaatcaatttgtcggattcacacgtgataatcaaatacggtgaggcattcctattgggcgcccaaatacagcctcttcccaccgcatccactcattttattcctgatccggtcaggacgcgcaagctattgatgaataaaaaagaattaaaccatctcataggaagtgttgaaaggcaaggctataccatagtccctctttctttgtattggaaaaaaaataaaattaaaataaaaattgctctggccaaaggaaaaaaagagcatgacaaaagagacacgatcaaagacagagaatggc

SEQ ID NO: 66 - DNA, 618 bp, Acinetobacter baumannii
tgatatgtgggaaaaaacttcaccttggcatcagtttacggcacaatagggacaattgtggaagtttgaattatggcgaaagcaacagtagtaaagaaacataatggcggaaccatcgcacaaaacaaacgtgcccgtcatgattattttatcgaagaaaaatttgaagctggcatgtctttactaggctgggaagtaaaatctttacgtgccggtcgtatgagtttgacagaaagttatgtcatttttaaaaatggtgaagcattcttatttggtgctcagattcaaccactcctttctgcatctacacatattgtgccggaagctacacgtacacgaaaattattattatctcgtcgtgaacttgaaaagcttatgggtgcggtgaaccaaaaaggttattcttgcgttccattagcatgttactggaaaggtcatctggttaagcttgaaattgcactcgtgaaaggtaaacaacttcacgataaacgagcgactgaaaaagaacgtgactggcaacgtgataaagcacgtatatttcataagtaatagactaaaaagccctttatagaggcttttttattttccactaatttaatctatataaaagcccagcaa

SEQ ID NO: 67 - DNA, 619 bp, Acinetobacter baumannii
tgatatgtgggaaaaaacttcaccttggcatcagtttacggcacaatagggacaattgtggaagtttgaattatggcgaaagcaacagtagtaaagaaacataatggcggaaccattgcacaaaacaaacgtgcccgtcatgattattttatcgaagaaaaatttgaagctggcatgtctttactaggctgggaagtaaaatctttacgtgccggtcgtatgagtttgacagaaagttatgtcatttttaaaaatggtgaagcattcttatttggtgctcagattcaaccactcctttctgcatctacacatattgtgccggaagctacacgtacacgaaaattattattatctcgtcgtgaacttgaaaagcttatgggtgcagtgaaccaaaaaggttattcgtgcgttccattagcatgttactggaaaggtcatctggttaagcttgaaattgcactcgtgaaaggtaaacaacttcacgataaacgagcaactgaaaaagaacgtgactggcaacgtgataaagcacgtatatttcataagtaatagactaaaaagcctctttatagaggcttttttatttttcactaatttaatctatataaaagcccagcaa

SEQ ID NO: 68 - DNA, 619 bp, Acinetobacter baumannii; identical to SEQ ID NO: 67

SEQ ID NO: 69 - DNA, 619 bp, Acinetobacter baumannii
atatgtgggaaaaaacttcaccttggcatcagtttacggcacaatagggacaattgtggaagtttgaattatggcgaaagcaacagtagtaaagaaacataatggcggaaccattgcacaaaacaaacgtgcccgtcatgattattttatcgaagaaaaatttgaagctggcatgtctttactaggctgggaagtaaaatctttacgtgccggtcgtatgagtttgacagaaagttatgtcatttttaaaaatggtgaagcattcttatttggtgctcagattcaaccactcctttctgcatctacacatattgtgccggaagctacacgtacacgaaaattattattatctcgtcgtgaacttgaaaagcttatgggtgcggtgaaccaaaaaggttattcgtgcgttccattagcatgttactggaaaggtcatctggttaagcttgaaattgcactcgtgaaaggtaaacaacttcacgataaacgagcaactgaaaaagaacgtgactggcaacgtgataaagcacgtatatttcataagtaatagactaaaaagcctctttatagaggcttttttatttttcactaatttaatctatataaaagcccagcaata

SEQ ID NO: 70 - DNA, 619 bp, Acinetobacter baumannii
tgatatgtgggaaaaaacttcaccttggcatcagtttacggcacaatagggacaattgtggaagtttgaattatggcgaaagcaacagtagtaaagaaacataatggcggaaccatcgcacaaaacaaacgtgcccgtcatgattattttatcgaagaaaaatttgaagctggcatgtctttactaggctgggaagtaaaatctttacgtgccggtcgtatgagtttgacagaaagttatgtcatttttaaaaatggtgaagcattcttatttggtgctcagattcaaccactcctttctgcatctacacatattgtgccggaagctacacgtacacgaaaattattattatctcgtcgtgaacttgaaaagcttatgggtgcggtgaaccaaaaaggttattcgtgcgttccattagcatgttactggaaaggtcatctggttaagcttgaaattgcactcgtgaaaggtaaacaacttcacgataaacgtgcgactgaaaaagaacgtgactggcaacgtgataaagcacgtatatttcataagtaatagactaaaaagcctctttatagaggcttttttatttttcactaatttaatctatataaaagcccagcaa

SEQ ID NO: 71 - DNA, 619 bp, Acinetobacter baumannii
tgatatgtgggaaaaaacttcaccttggcatcagtttacggcacaatagggacaattgtggaagtttgaattatggcgaaagcaacagtagtaaagaaacataatggcggaaccatcgcacaaaacaaacgtgcccgtcatgattattttatcgaagaaaaatttgaagctggcatgtctttactaggctgggaagtaaaatctttacgtgccggtcgtatgagtttgacagaaagttatgtcatttttaaaaatggtgaagcattcttatttggtgctcagattcaaccactcctttctgcatctacacatattgtgccggaagctacgcgtacacgaaaattattattatctcgtcgtgaacttgaaaagcttatgggtgcggtgaaccaaaaaggttattcgtgcgttccattagcatgttactggaaaggtcatctggttaagcttgaaattgcactcgtgaaaggtaaacaacttcacgataaacgagcgactgaaaaagaacgtgactggcaacgtgataaagcacgtatatttcataagtaatagactaaaaagcctctttatagaggcttttttatttttcactaatttaatctatataaaagcccagcaa

SEQ ID NO: 72 - DNA, 619 bp, Acinetobacter baumannii
cattaaaatgaaaaaacttcacctcggtcgttgtttaaggcacaataagcataactttggaattttaagattatgtcgaaagcagtagtagttaaaaaaaataatggcggtaccattgcgcagaataaacgcgcccgacacgattattttattgaagaaaaatttgaagcaggtatgtctttgcaaggctgggaagtaaaatccttgcgtgcaggtcgtatgagccttaccgaaagctatatcatctttaaaaatggtgaagcctacctatttggtgctcaaattcaaccgttgcttaccgcatcgagccatgttgtgcctgaagccacacggacacgtaaattactactgtcacgtcgtgaaattggtcaactactaggtgctgtcaatcagaaaggttattcgtgtgtacctttggcatgttactggaaaggtcacttggtcaagctcgaaattgcactggtgaaagggaaacagttacatgataagcgtgcaaccgaaaaagatcgtgactggcaacgtgacaaagcacggattatgcataagtaatttatacaaaaagcctttactaaggctttttgtttgattgtttaatgcaaacggtaaagtaacccaccga

SEQ ID NO: 73 - DNA, 619 bp, Acinetobacter baumannii
tgatatgtgggaaaaaacttcaccttggcatcagtttacggcacaataggggcaattgtggaagtttgaattatggcgaaagcaacagtagtaaagaaacataatggcggaaccatcgcacaaaataaacgtgcccgtcatgattattttatcgaagaaaaatttgaagctggcatgtctttactcggctgggaagtaaagtctttacgtgctggtcgtatgagtttgacagaaagttatgtcatttttaaaaacggtgaagcatttttatttggtgcgcaaattcaaccgctcctttctgcatctacacatatcgtgccggaagctacacgtacacgtaaattattattatctcgtcgtgaacttgaaaagcttatgggtgcagtgaaccaaaaaggttattcgtgcgttccattagcatgttactggaaaggtcatctggtcaagcttgaaattgcactcgtgaaaggtaaacaactccacgataaacgtgcgactgaaaaagaacgtgactggcaacgtgataaagcccgtatatttcataaataatagactaaaaagcctctataaagaggcttttttattttttactaatttaatctatataaaagtccagcaa

SEQ ID NO: 74 - DNA, 572 bp, Acinetobacter baumannii
aaaaacttcaccttagcatcagtttacggcacaataggggcaattgtggaagtttgaattatggcgaaagcaacagtagtgaaaaaacataatggtggaaccatcgcacaaaacaaacgtgcccgccatgattattttatcgaagaaaaatttgaagctggtatgtctttactcggctgggaagtaaagtctttacgtgctggtcgcatgagtttgacagaaagttatgtcatttttaagaatggtgaagcgtttttatttggtgcacaaattcaaccgctcctttcagcatctactcatgtagtacctgaagctacacgtacacgtaaattattattatcacgccgagaactagaaaagctaacaggttcagttaaccaaaaaggttactcatgtgttcctttagcatgttactggaaaggtcacttggttaaacttgaaatcgcgcttgtgaaaggtaaacagcttcacgacaaacgtgcgactgaaaaagatcgcgattggcagcgtgataaagctcgtatatttcataagtaattaaataaaaagcctctttttagaggcttttttat

SEQ ID NO: 75 - DNA, 477 bp, Acinetobacter calcoaceticus
atggcgaaagcaacagtagtaaagaaacataatggcggaaccatcgcacaaaataaacgtgcccgtcatgattattttatcgaagaaaaatttgaagctggtatgtctttactcggctgggaagtaaagtctttacgtgctggtcgcatgagtttgacagaaagttatgtcatttttaagaatggtgaagcgtttttatttggtgcacaaattcaaccgctcctttcggcatctactcatgtagtacctgaagctacacgtacacgtaaattattattatcacgccgagaactagaaaagctaacgggttcagtgaaccaaaaaggttactcatgtgttcctttggcatgttattggaaaggtcacttggtgaagcttgaaatcgcgcttgtgaaaggtaaacagcttcacgacaaacgtgcgactgaaaaagatcgcgattggcagcgtgataaagctcgtatatttcataagtaa

SEQ ID NO: 76 - DNA, 619 bp, Acinetobacter calcoaceticus
gacgtgcaggaaaaacttcaccttagcatcagtttacggcacaataggggcaattgtggaagtttgaattatggcgaaagcaacagtagtaaagaaacataatggcggaaccatcgcacaaaataaacgtgcccgtcatgattattttatcgaagaaaaatttgaagctggtatgtctttactcggctgggaagtaaagtctttacgtgctggtcgcatgagtttgacagaaagttatgtcatttttaagaatggtgaagcgtttttatttggtgcacaaattcaaccgctcctttcggcatctactcatgtagtacctgaagctacacgtacacgtaaattattattatcacgccgagaactagaaaagctaacgggttcagtgaaccaaaaaggttactcatgtgttcctttggcatgttattggaaaggtcacttggtgaagcttgaaatcgcgcttgtgaaaggtaaacagcttcacgacaaacgtgcgactgaaaaagatcgcgattggcagcgtgataaagctcgtatatttcataagtaattaaataaaaagcctctttttagaggcttttttatatcgcggaatttattaatttaatctatataagagtcc

SEQ ID NO: 77 - DNA, 572 bp, Acinetobacter calcoaceticus; identical to SEQ ID NO: 74

SEQ ID NO: 78 - DNA, 614 bp, Acinetobacter calcoaceticus
aaaaacttcaccttagcatcagtttacggcacaataggcataattgtggaagtttgaattatggcgaaagcaacagtagtaaagaaacataatggcggaacaatcgcacaaaataaacgtgcccgtcatgattattttatcgaagaaaaatttgaagcgggcatgtcacttcaaggttgggaagtaaaatccttacgtgctgggcgcatgactttgacggaaagttatgtcattttcaagaatggcgaagcatttttacttggctcacaaattcagcctttattatcggcttcgacccatgtggtacctgaagcaacacgcacccgtaagttattgctctcccgacgtcagcttgaacacctaatgggtgcagttaaccaaaaaggttactcatgtgttcctttggcgtgttactggaaaggtcacttggttaaacttgaaattgcgcttgtgaaaggtaaacagcttcacgacaaacgtgcaactgaaaaagaccgcgactggcagcgtgataaagctcgtatatttcataaataatttaataaaaaagcctctttttagaggctttttatatttttgactttattaatttaatctatataaaagcccagcaa

SEQ ID NO: 79 - DNA, 539 bp, Acinetobacter calcoaceticus
aaaaacttcaccttagcatcagtttacggcacaataggcataattgtggaagtttgaattatggcgaaagcaacagtagtaaagaaacataatggcggaacaatcgcacaaaataaacgtgcccgtcatgattattttatcgaagaaaaatttgaagcaggcatgtcacttcaaggttgggaagtaaaatccttacgtgctgggcgtatgactttgacggaaagttatgtcattttcaagaatagcgaagcatttttacttggttcacaaattcagcctttattatcggcttcgacccatgtggtacctgaagcaacacgtacccgtaagttattgctctcccgccgtcagcttgaacacctgatgggtgcagttaaccaaaaaggttactcgtgcgttcctttggcgtgttactggaaaggtcacttggttaaacttgaaattgcacttgtgaaaggtaaacaacttcacgacaaacgtgcaactgaaaaagaccgtgactggcaacgtgataaagctcgtatatttcataagtaata

SEQ ID NO: 80 - DNA, 570 bp, Acinetobacter calcoaceticus
aaaaacttcaccttagcatcagtttacggcacaataggcataattgtggaagtttgaattatggcgaaagcaacagtagtgaaaaaacacaatggcggaacaatcgcacaaaacaaacgtgcccgtcatgattattttatcgaagaaaaatttgaagcaggcatgtcacttcaaggttgggaagtaaaatccttacgtgctggacgtatgactttgactgaaagttatgtgattttcaaaaatggcgaagcatttttacttggctcacaaattcagcctttattatcagcttcgactcatgttgtacctgaagcaacacgtacccgtaagttattgctctcccgacgtcagcttgaacacctaatgggtgcagttaaccagaaaggttactcatgcgttcctttagcgtgttactggaagggtcatttagtcaaactagagattgcacttgtgaagggtaaacagcttcatgacaaacgtgcaactgaaaaagaccgtgactggcaacgtgataaagctcgtatatttcataagtaataaaataaaagcctcttttcagaggctttttta

SEQ ID NO: 81 - DNA, 477 bp, Acinetobacter calcoaceticus
atggcgaaagcaacagtagtgaaaaaacacaatggcggaacaatcgcacaaaataaacgtgcccgtcatgattattttattgaagaaaaatttgaagctggtatgtcacttcaaggttgggaagtaaaatccttacgtgctgggcgtatgactttgacggaaagttatgtcattttcaagaatagcgaagcatttttacttggttcacaaattcagcctttattatcggcttcgacccatgtggtacctgaagcaacacgtacccgtaagttattactctccagacgtcagcttgaacacctaatgggtgcagttaaccaaaaaggttactcatgcgttcctttggcgtgttactggaaaggtcatttagtcaaacttgaaattgcacttgtgaaaggtaaacaacttcacgacaaacgtgcaaccgaaaaagaccgtgactggcaacgtgataaagctcgtatatttcataagtaa

SEQ ID NO: 82 - DNA, 539 bp, Acinetobacter calcoaceticus
aaaaacttcaccttagcatcagtttacggcacaataggcataattgtggaagtttgaattatggcgaaagcaacagtagtgaaaaaacacaatggcggaacaatcgcacaaaataaacgtgcccgtcatgattattttatcgaagaaaaatttgaagcgggtatgtcacttcaaggttgggaagtaaaatccttacgcgctgggcgcatgactttgacggaaagttatgtcattttcaagaatggcgaagcatttttacttggctcacaaattcagcctttattatcggcttcgacccatgtggtacctgaagcaacacgcacccgtaagttattactctcccgacgtcagcttgaacacctaatgggtgcagttaaccaaaaaggttactcatgcgttcctttggcgtgttactggaaaggtcatttagtcaaacttgaaattgcgcttgtgaaaggtaaacaacttcacgacaaacgtgcaactgaaaaagaccgtgactggcaacgtgataaagctcgtatatttcataagtaata

SEQ ID NO: 83 - DNA, 539 bp, Acinetobacter calcoaceticus
aaaaacttcaccttagcatcagtttacggcacaataggcataattgtggaagtttgaattatggcgaaagcaacagtagtgaaaaaacacaatggcggaacaatcgcacaaaataaacgtgcccgtcatgattattttatcgaagaaaaatttgaagcgggtatgtcacttcaaggttgggaagtaaaatccttacgtgctgggcgtatgactttgacggaaagttatgtcattttcaagaatggcgaagcatttttacttggctcacaaattcagcctttattatcggcttcgacccatgtggtacctgaagcaacacgcacccgtaagttattgctctcccgacgtcagcttgaacacctaatgggcgcagttaaccaaaaaggttactcatgtgttcctttggcgtgttactggaaaggtcacttggttaaacttgaaattgcgcttgtgaaaggtaaacagcttcacgacaaacgtgcaactgaaaaagaccgtgactggcaacgtgataaagctcgtatatttcataagtaata

SEQ ID NO: 84 - DNA, 539 bp, Acinetobacter calcoaceticus; identical to SEQ ID NO: 83

SEQ ID NO: 85 - DNA, 539 bp, Acinetobacter calcoaceticus
aaaaacttcaccttagcatcagtttacggcacaataggcataattgtggaagtttgaattatggcgaaagcaacagtagtgaaaaaacacaatggcggaacaatcgcacaaaataaacgtgcccgtcatgattattttatcgaagaaaaatttgaagcgggtatgtcacttcaaggttgggaagtaaaatccttacgtgctgggcgtatgactttgacggaaagttatgtcattttcaagaatggcgaagcatttttacttggctcacaaattcagcctttattatcggcttcaactcatgtggtacctgaagcaacacgcacccgtaagttattgctctcccgacgtcagcttgaacacctaatgggtgcagttaaccaaaaaggttactcatgcgttcctttggcgtgttactggaaaggtcatttagtcaaactagaaattgcgcttgtgaagggtaaacaacttcatgacaaacgtgcaactgaaaaagaccgtgactggcaacgtgataaagctcgtatatttcataagtaata

SEQ ID NO: 86 - DNA, 465 bp, Acinetobacter nosocomialis
agttgtaaagaaacataatggcggaaccatcgcacaaaataaacgtgcccgtcatgattattttatcgaagaaaaatttgaagctggcatgtctttactcggctgggaagtaaagtctttacgtgctggtcgtatgagtttgacagaaagttatgtcatttttaaaaacggtgaagcatttttatttggtgcacaaattcaaccgctcctttctgcatctacacatatcgtgccggaagctacacgtacacgtaaattattattatctcgtcgtgaacttgaaaagcttatgggtgcagtgaaccaaaaaggttattcgtgcgttccattagcgtgttactggaaaggtcatctagtcaagcttgaaattgcactcgtgaaaggtaaacaactccacgataaacgtgcaactgaaaaagaacgtgactggcaacgtgataaagctcgtatatttcataaataata

SEQ ID NO: 87 - DNA, 465 bp, Acinetobacter nosocomialis; identical to SEQ ID NO: 86

SEQ ID NO: 88 - DNA, 619 bp, Acinetobacter nosocomialis
tgatatgtgggaaaaaacttcaccttggcatcagtttacggcacaatagggacaattgtggaagtttgaattatggcgaaagcaacagtagtaaagaaacataatggcggaaccatcgcacaaaataaacgtgcccgtcatgattattttatcgaagaaaaatttgaagctggcatgtctttactcggctgggaagtaaagtctttacgtgctggtcgtatgagtttgacagaaagttatgtcatttttaaaaacggtgaagcatttttatttggtgcacaaattcaaccgctcctttctgcatctacacatatcgtgccggaagctacacgtacacgtaaattattattatctcgtcgtgaacttgaaaagcttatgggtgcagtgaaccaaaaaggttattcgtgcgttccattagcgtgttactggaaaggtcatctggtcaagcttgaaattgcactcgtgaaaggtaaacaactccacgataaacgtgcgactgaaaaagaacgtgactggcaacgtgataaagcccgtatatttcataaataatagactaaaaagcctctataaagaggcttttttattttttactaatttaatctatataaaagtccagcaa

SEQ ID NO: 89 - DNA, 619 bp, Acinetobacter nosocomialis
tgatatgtgggaaaaaacttcaccttggcatcagtttacggcacaataggggcaattgtggaagtttgaattatggcgaaagcaactgtagtaaagaaacataatggcggaaccatcgcacaaaataaacgtgcccgtcatgattattttatcgaagaaaaatttgaagctggcatgtctttactcggctgggaagtaaagtctttacgtgctggtcgtatgagtttgacagaaagttatgtcatttttaaaaacggtgaagcatttttatttggtgcacaaattcaaccgctcctttctgcatctacacatatcgtgccggaagctacacgtacacgtaaattattattatctcgtcgtgaacttgaaaagcttatgggtgcagtgaaccaaaaaggttattcgtgcgttccattagcatgttactggaaaggtcatctggtcaagcttgaaattgcactcgtgaaaggtaaacaactccacgataaacgtgcgactgaaaaagaacgtgactggcaacgtgataaagcccgtatatttcataaataatagactaaaaagcctctataaagaggcttttttattttttactaatttaatctatataaaagtccagcaa

SEQ ID NO: 90 - DNA, 533 bp, Acinetobacter nosocomialis
agttgtaaagaaacataatggcggaaccatcgcacaaaataagcgtgcccgtcatgattattttatcgaagaaaaatttgaagctggcatgtctttactcggctgggaagtaaagtctttacgtgccggtcgtatgagtttgacagaaagttatgtcatttttaaaaacggtgaagcatttttatttggtgcacaaattcaaccgcttctttctgcatctacacatattgtgccggaggctacacgtacacgtaaattattattatctcgtcgtgaacttgaaaagcttatgggtgcagtgaaccaaaaaggttattcgtgcgttccattagcgtgttactggaaaggtcatctggtcaagcttgaaattgcactcgtgaaaggtaaacaactccacgataaacgtgcaactgaaaaagaacgtgactggcaacgtgataaagcccgtatatttcataaataatagactaaaaagcctctataaagaggcttttttattttttactaatttaatctatataaaagtccagcaa

SEQ ID NO: 91 - DNA, 533 bp, Acinetobacter nosocomialis; identical to SEQ ID NO: 90

SEQ ID NO: 92 - DNA, 572 bp, Acinetobacter genomosp.
aaaaacttcaccttagcatcagtttacggcacaataggggcaattgtggaagtttgaattatggcgaaagcaacagtagtaaagaaacataatggcggaaccatcgcacaaaataaacgtgcccgtcatgattattttatcgaagaaaaatttgaagctggtatgtctttactcggctgggaagtaaagtctttacgtgctggtcgcatgagtttgacagaaagttatgtcatttttaagaatggtgaagcgtttttatttggtgcacaaattcaaccgctcctttcggcatctactcatgtagtacctgaagctacacgtacacgtaaattattattatcacgccgagaactagaaaagctaacgggttcagttaaccaaaaaggttactcatgtgttcctttagcatgttattggaaaggtcacttggtgaagcttgaaatcgcgcttgtgaaaggtaaacagcttcacgacaaacgtgcgactgaaaaagatcgcgattggcagcgtgataaagctcgtatatttcataagtaattaaataaaaagcctctttttagaggcttttttat

SEQ ID NO: 93 - DNA, 613 bp, Acinetobacter genomosp.
aaaaacttcaccttagcatcagtttacggcacaataggcataattgtggaagtttgaattatggcgaaagcaacagtagtaaagaaacataatggcggaaccatcgcacaaaacaaacgtgcccgccatgattattttatcgaagaaaaatttgaagctggtatgtctttactcggttgggaagtaaagtctttacgtgctggtcgcatgagtttgacagaaagttatgtcatttttaagaatggtgaagcgtttttatttggtgcacaaattcaaccgctcctttcagcatctactcatgtagtacctgaagctacacgtacacgtaaattattattatcgcgccgagaactagaaaagctaacaggttcagttaaccaaaaaggttactcatgtgttcctttggcatgttactggaaaggtcacttggttaaacttgaaatcgcgcttgtgaaaggtaaacagcttcacgacaaacgtgcgactgaaaaagatcgcgattggcagcgtgataaagctcgtatatttcataagtaattaaataaaaagcctctttttagaggctttttatatcgcggaatttattaatttaatctatataagagtccagcaa

SEQ ID NO: 94 - DNA, 619 bp, Acinetobacter oleivorans
ttcatgtgcaggaaaaacttcaccttagcatcagtttacggcacaataggcataattgtggaagtttgaattatggcgaaagcaacagtagtaaagaaacataatggcggaacaatcgcacaaaataagcgtgcccgtcatgattattttatcgaagaaaaatttgaagcaggcatgtcacttcaaggttgggaagtaaaatccttacgtgctgggcgtatgactttgacggaaagttatgtcattttcaaaaatggcgaagcatttttacttggttcacaaattcagcctttattatcggcttcgacccatgttgtacctgaggcaacacgtacccgtaaactattgctctcccgacgtcagcttgaacatctaatgggtgcagttaaccagaaaggctactcatgtgttcctttagcgtgttattggaaaggtcatttagtcaaactggagattgcacttgtgaagggtaaacagcttcatgacaaacgtgcaaccgaaaaagaccgtgactggcaacgtgataaagctcgtatatttcataagtaataaaacaaaagcctcttttcagaggcttttttacgtcgtgaagttcattagtttaatctgtataaaagtc

SEQ ID NO: 95 - DNA, 615 bp, Acinetobacter pittii
aaaaacttcaccttagcatcagtttacggcacaatagaggcaattgtggaagtttgaattatggcgaaagcaacagtagtaaagaaacataatggcggaaccatcgcacaaaataaacgtgcccgtcatgattattttatcgaagaaaaatttgaagctggtatgtctttactcggctgggaagtaaagtctttacgtgctggtcgcatgagtttgacagaaagttatgtcatttttaagaatggtgaagcgtttttatttggtgcacaaattcaaccgctcctttcggcgtctactcatgtagtacctgaagctacacgtacacgtaaattattattatcacgccgagaactagaaaagctaacaggttcagtgaaccaaaaaggttactcatgtgttcctttagcatgttattggaaaggtcacttggttaaacttgaaattgctctggtgaaaggtaaacagcttcatgacaaacgtgcgactgaaaaagatcgcgattggcaacgtgataaagctcgtatatttcataagtaattaaataaaaagcctctttcttagaggcttttttacatcgtaaagtttattaatttaatctatataaaagaccagcaa

SEQ ID NO: 96 - DNA, 572 bp, Acinetobacter pittii
aaaaacttcaccttagcatcagtttacggcacaataggggcaattgtggaagtttgaattatggcgaaagcgacagtagtgaaaaaacataatggcggaaccatcgcacaaaacaaacgtgcccgccatgattattttatcgaagaaaaatttgaagctggtatgtctttactaggctgggaagtaaagtctttacgtgctggtcggatgagcttgacagaaagttatgtcatttttaagaatggtgaagcgtttttatttggtgcacaaattcaaccgctcctttcagcatctactcatgtagtacctgaagctacacgtacacgtaaattattattatcacgccgagaactagaaaagctaacaggttcagttaaccaaaaaggttactcatgtgttcctttggcatgttactggaaaggtcacttggttaaacttgaaatcgcgcttgtgaaaggtaaacaacttcacgacaaacgtgcgactgaaaaagatcgcgattggcagcgtgataaagctcgtatatttcataagtaattaaataaaaagcctctttttagaggcttttttat

SEQ ID NO: 97 - DNA, 572 bp, Acinetobacter pittii; identical to SEQ ID NO: 74

SEQ ID NO: 98 - DNA, 572 bp, Acinetobacter pittii; identical to SEQ ID NO: 92

SEQ ID NO: 99 - DNA, 572 bp, Acinetobacter pittii
aaaaacttcaccttagcatcagtttacggcacaataggggcaattgtggaagtttgaattatggcgaaagcgacagtagtgaaaaaacataatggcggaaccatcgcacaaaacaaacgtgcccgccatgattattttatcgaagaaaaatttgaagctggtatgtctttactcggctgggaagtaaagtctttacgtgctggtcggatgagcttgacagaaagttatgtcatttttaagaatggtgaagcgtttttatttggtgcacaaattcaaccgctcctttcagcatctactcatgtagtacctgaagctacacgtacacgtaaattattattatcacgccgagaactagaaaagctaacaggttcagttaaccaaaaaggttactcatgtgttcctttagcatgttactggaaaggtcacttggttaaacttgaaatcgcgcttgtgaaaggtaaacaacttcacgacaaacgtgcgactgaaaaagatcgcgattggcagcgtgataaagctcgtatatttcataagtaattaaataacaagcctctttttagaggcttttttat

SEQ ID NO: 100 - DNA, 539 bp, Acinetobacter pittii
aaaaacttcaccttagcatcagtttacggcacaataggggcaattgtggaagtttgaattatggcgaaagcaacagtagtaaagaaacataatggcggaaccatcgcacaaaacaaacgtgcccgccatgattattttatcgaagaaaaatttgaagctggtatgtctttactcggctgggaagtaaagtctttacgtgctggtcgcatgagtttgacagaaagttatgtcatttttaagaatggtgaagcgtttttatttggtgcacaaattcaaccgctcctttctgcctctactcatgtagtacctgaagctacacgtacacgtaaattattattatcacgccgagaactagaaaagttaacaggttcagttaaccaaaaaggttactcatgtgttcctttggcatgttactggaaaggtcacttggttaaacttgaaattgcccttgtgaaaggtaagcagcttcatgacaaacgtgcgactgaaaaagatcgcgattggcagcgtgataaagctcgtatatttcataagtaata

SEQ ID NO: 101 - DNA, 517 bp, Acinetobacter junii
tttacggcacaatagatgcaattgtggaagtttgaattatggcgcaagcaacagttgtaaaaaaacataatggtggcacgattgctcaaaataaaagagcgcgtcacgattactttatcgaagaaaaatttgaagcaggcatgtcacttcagggttgggaagtaaaatccttacgtgctggacgtatgaccttgtctgaaagttatgtcatttttaaaaatggtgaagcctttttatttggttcacagattcagcctttattgtctgcatcaacccatgtcgtacctgaatcgacacgtacacgaaagttattattatctcgtcgtgaactagaaaagttactaggtgctgtgaaccaaaaaggttattcatgtgttcctttagcctgctattggaaaggtcacttggttaagctcgaaattgcgttggtcaaaggtaagcaattacatgacaaacgtgctacggaaaaagaccgtgattggcagcgtgataaagcacgtatgttgcataaataata

SEQ ID NO: 102 - DNA, 517 bp, Acinetobacter junii
tttacggcacaatagatgcaattgtggaagtttgaattatggcgcaagcaacagttgtaaaaaaacataatggtggcacgattgctcaaaataaaagagcgcgtcacgattattttatcgaagaaaaatttgaagcaggcatgtcacttcagggttgggaagtaaaatccttacgcgctggacgtatgaccttgtctgaaagttatgtcatttttaaaaatggtgaagcctttttatttggttcacagattcagcctttattgtctgcatcaacccatgtcgtacctgaatcaacacgtacacgaaagttattattatctcgtcgtgaactagaaaagttactaggcgcagtgaaccaaaaaggttattcatgtgttcctttagcctgctattggaaaggtcacttggttaagctcgaaattgcgttggtcaaaggtaagcaattacatgacaaacgtgctacggaaaaagaccgtgattggcagcgtgataaagcacgtatgttgcataaataata

SEQ ID NO: 103 - DNA, 517 bp, Acinetobacter junii
tttacggcacaatagatgcaattgtggaagtttgaattatggcgcaagcaacagttgtaaaaaaacataatggtggcacgattgctcagaataaaagagcgcgtcacgattactttatcgaagaaaaatttgaagcaggcatgtcacttcagggttgggaagtaaaatccttacgtgctggacgtatgacattgtctgaaagttatgtcatttttaaaaatggtgaagcctttttatttggttcacagattcagcctttattgtctgcatcaacccatgtcgtacctgaatcgacacgtacacgaaagttattattatctcgtcgtgaactagaaaagttactaggcgcagtgaaccaaaaaggttattcatgtgttcctttagcctgctattggaaaggtcacttggttaagctcgaaattgcgttggtcaaaggtaagcaattacatgacaaacgtgctacggaaaaagaccgtgattggcagcgtgataaagcacgtatgttgcataaataata

SEQ ID NO: 104 - DNA, 517 bp, Acinetobacter junii; identical to SEQ ID NO: 103

SEQ ID NO: 105 - DNA, 517 bp, Acinetobacter junii
tttacggcacaatagatgcaattgtggaagtttgaattatggcgcaagcaacagttgtaaaaaaacataatggtggcacgattgctcagaataaaagagcgcgtcacgattactttatcgaagaaaaatttgaagcaggcatgtcacttcagggttgggaagtaaaatccttacgtgctggacggatgactttgtctgaaagttatgtcatttttaaaaatggtgaagcctttttatttggttcacagattcagcctttattgtctgcatcaacccatgtcgtacctgaatcaacacgtacacgaaagttattattatctcgtcgcgaactagaaaagttactaggcgcagtgaaccaaaaaggttattcatgtgttcctttagcctgctattggaaaggtcacttggttaagctcgaaattgcgttggtcaaaggtaagcaattacatgacaaacgtgctacggaaaaagaccgtgattggcagcgtgataaagcacgtatgttgcataaataata

SEQ ID NO: 106 - DNA, 517 bp, Acinetobacter junii; identical to SEQ ID NO: 105

SEQ ID NO: 107 - DNA, 546 bp, Acinetobacter gyllenbergii
tttacggcacaatagagccaattgtggaagtttaaattatggcgcaagcaacagttgtaaaaaaacataatggtggcacgattgctcaaaataaaagagcgcgccacgattactttatcgaagaaaaatttgaagcaggcatgtccctacaaggttgggaagtaaaatccctacgtgctgggcgtatgagcttgactgaaagttatgtcatttttaaaaatggtgaagcttttttattgggctcacaaattcagcccttgttgtctgcctcaactcatgtggttccagaagcaacacgtacgcgtaaattactgctctctcgtcgtgagctagaaaagcttttgggtgcagtgaatcaaaaaggctattcatgtgtacctttggcatgttattggaaaggccatttggtcaaacttgaaattgcactggtgaaaggtaagcaattacatgacaagcgtgccactgaaaaagaccgtgactggcaacgtgataaatctcgtctgctgcataagtaataaaaaaacctccaattggaggtttttttat

SEQ ID NO: 108 - DNA, 546 bp, Acinetobacter gyllenbergii; identical to SEQ ID NO: 107

SEQ ID NO: 109 - DNA, 517 bp, Acinetobacter beijerinckii
tttacggcacaataggcataattgtggaagtttgaattatggcgaaagcaactgtagttaaaaaaaataatggtggaacgattgctcaaaacaaaagagcgcgtcacgattactttattgaagaaaaaattgaagctggtatgtctttacaaggctgggaagtgaaatcacttcgtgccggtcgtatgactctgactgaaagctatgtcatttttaaaaatggtgaagcatttttactgggttcacaaattcagcctttattgtcagcatcaagtcatgtggttcctgaggcaactcgtacacgtaagttactactttctcgccgtgagatagatagactaatgggcgcagtgaatcagaaaggttattcatgtgttcctctggcatgttattggaaaggtcctttggttaaactagaaattgccatggttaaaggtaaacagttacacgataaacgtgcaactgaaaaagatcgtgactggcaacgagataaatcacgtatgttgcataaataata

SEQ ID NO: 110 - DNA, 517 bp, Acinetobacter beijerinckii
tttacggcacaataggcataattgtggaagtttgaattatggcgaaagcaactgtagttaaaaaaaataatggtggaacgattgctcaaaacaaaagagcgcgtcacgattactttattgaagaaaaaattgaagctggtatgtctttacaaggctgggaagtgaagtcacttcgtgccggtcgtatgacgctgactgaaagctatgtcatttttaaaaatggtgaagcatttttactgggttcacaaattcagcctttattatcagcatcaagtcatgtggttcctgaggcaactcgtacacgtaagttactactttctcgccgtgagatagatagactaatgggcgcagtgaatcagaaaggttattcatgtgttcctctggcatgttattggaaaggtcctttggttaaactagaaattgccatggttaaaggtaaacagttacacgataaacgtgcaactgaaaaagatcgtgactggcaacgagataaatcacgtatgttgcataaataata

SEQ ID NO: 111 - DNA, 531 bp, Acinetobacter brisouii
aaaagcttcaccttgggaaaagtttgcggcacaatagatacagttttggaatgatttaattatggcgaaagcaactgtagtcaagaaaaataatggcggaactattgcacaaaataagcgtgcccgtcatgattattttatcgaagaaaaatttgaagcgggtctttccctacagggttgggaagtcaaatccttgcgtgctgggcgtatgagtctggttgagagctatattatttttaaaaataatgaagcgtttttatttggcgcacagattcagccactcttgtctgcctcaactcatgtcgtacccgaagccactcgcactcgcaaactattactgtcacgccgtgaactggaacagctcacaggcgcagtaaatcaaaaaggttacacttgtgtacctttagcatgttactggaaaggacatttggcgaaactggaaattgcgctggtaaaaggtaagcaactccatgataaacgcgctactgaaaaagaccgcgactggcaacgtgataaagcccgtatttttca

SEQ ID NO: 112 - DNA, 574 bp, Acinetobacter lwoffii
gaaaaaacttcaccttaaccatgctttaaggcacaataggtacattgttggaagtaattgattatggcgaaagcaactgtagttaaaaaaaataccagcgggacgattgcacagaataaacgtgcacgtcacgactattttattgaagaaaaatttgaagctggcctgtcactgcaaggctgggaagtgaaatcattacgtgcaggtcgtatgacgctgtctgagagttatatcacctttaaaaatggtgaagctttcctgttcggtgctcaaattcagcctttactcagtgcatctacgcacattgttcctgaagcgacccgtacccgtaagttactgttgaaccgtcgtgaactggataagctactcggcgcagtgaatcaaaaaggttattcgtgtgttccacttgttgcttattggaaaggaccacgtgcgaaattagaaatcgctttagtgaaaggcaaacagctgcatgacaaacgtgccacggaaaaagaccgtgactggcaacgtgataaagcccgtattatgcataaataataaaaaacctcccatgtggaggttttttattatc

SEQ ID NO: 113 - DNA, 551 bp, Acinetobacter lwoffii
aaaaaacttcaccttatttctagttgcggtacaatagcagcacgtttggaagtatcagattatggcgaaagcatctattgtagtaaaaaaaaataatggcggtaccattgcactgaataaacgtgcccgccacgattattttattgaagagaaatttgaagcggggctgtcattaaagggctgggaagtcaaatcaatgcgtgccggtcgtatgaccattgtagaaagctatattacctttaaaaatggtgaagctttcctgtttggtgcgcaagttcagcctttgctgagtgcttcaacacacgtggtgcctgaagcgacccgtacccgaaaactgttgttgaatcgccgtgaaattgaaaagctgatgggcgcgattaaccagaaaggttattcctgcgtgccactggcctgttactggaaaggcccgcatgccaagctggaaattgcactggtcaaaggtaagcagcttcatgacaaacgtgccaccgagaaagaccgtgactggcaacgtgataaggcgcgaattttccataaataatggattaaaa

SEQ ID NO: 114 - DNA, 551 bp, Acinetobacter lwoffii
aaaaaacttcaccttatttctagttgcggtacaatagcagcacgtttggaagtatcagattatggcgaaagcatctattgtagtaaaaaaaaataatggcggtaccattgcactgaataaacgtgcccgccacgattattttattgaagagaaatttgaagcggggctttcattaaaaggctgggaagtcaaatcaatgcgtgctggtcgcatgaccatcgtagaaagttatattacctttaaaaatggtgaagcgttcttgtttggtgcacaggttcagcccttgttaagtgcttcgacccatgtggtgcctgaagcaacccgtacccgcaaactgttgctgaatcgccgtgaaattgaaaagttgatgggtgcgattaaccagaaaggttattcctgcgttccactggcctgctactggaaaggtccacatgccaagctggaaattgctctggtgaaaggtaagcagcttcatgacaaacgtgccaccgaaaaagaccgtgactggcaacgtgataaggcgcgaattttccataaataatggattaaaa

SEQ ID NO: 115 - DNA, 551 bp, Acinetobacter lwoffii; identical to SEQ ID NO: 114

SEQ ID NO: 116 - DNA, 552 bp, Acinetobacter lwoffii
aaaaaacttcaccttatttctagttgcggtacaatagcagcacgtttggaagtatcagattatggcgaaagcatctattgtagtaaaaaaaaataatggcggtaccattgcactgaataaacgtgcccgccacgattattttattgaagagaaatttgaagcggggctttcattaaaaggctgggaagtcaaatcaatgcgcgctggtcgcatgaccattgtagaaagttatattacctttaaaaatggtgaagcgttcttgtttggtgcacaggttcagcccttgttaagtgcttcgacccatgtggtgcctgaagcaacccgtacccgcaaactgttgctgaatcgccgtgaaattgaaaagttgatgggtgcgattaaccagaaaggttattcctgcgttccactggcctgctactggaaaggtccacatgccaagctggaaattgctctggtcaaaggtaagcagctccatgacaaacgtgccaccgaaaaagaccgtgactggcaacgtgataaagcacgaattttccataaataatggattaaaaa

SEQ ID NO: 117 - DNA, 550 bp, Acinetobacter lwoffii
aaaaaacttcaccttatttctagttgcggtacaatagcagcacgtttggaagtatcagattatggcgaaagcatctattgtagtaaaaaaaataatggcggtaccattgcactgaataaacgtgcccgccacgattattttattgaagagaaatttgaagcggggctttcattaaaaggctgggaagtcaaatcaatgcgcgctggtcgcatgaccattgtagaaagttatattacctttaaaaatggtgaagcgttcttgtttggtgcacaggttcagcccttgttaagtgcttcgacccatgtggtgcctgaagcaacccgtacccgcaaactgttgctgaatcgccgtgaaattgaaaagttgatgggtgcgattaaccagaaaggttattcctgcgttccactggcctgctactggaaaggtccacatgccaagctggaaattgctctggtcaaaggtaagcagcttcatgacaaacgtgccaccgaaaaagaccgtgactggcaacgtgataaagcgcgaattttccataaataatggattaaaa

SEQ ID NO: 118 - DNA, 551 bp, Acinetobacter lwoffii
aaaaaacttcaccttatttctagttgcggtacaatagcagcacgtttggaagtatcagattatggcgaaagcatctattgtagtaaaaaaaaataatggcggtaccattgcactgaataaacgtgcccgccacgattattttattgaagagaaatttgaagcggggctttcattaaaaggttgggaagtcaaatcaatgcgtgctggtcgcatgaccatcgtagaaagttatattacctttaaaaatggtgaagcgttcttgtttggtgcacaggttcagcccttgttaagcgcttcgacccatgtggtgcctgaagcaacccgtactcgcaagctgttgctgaatcgccgtgaaattgaaaagctgatgggtgcgattaaccagaaaggttattcctgcgtaccactggcgtgttactggaaaggtccacatgccaaactggaaattgccttggtgaaaggtaagcaactccatgacaaacgtgccaccgaaaaagaccgtgactggcaacgtgataaagcgcgaattttccataaataatggattaaaa

SEQ ID NO: 119 - DNA, 464 bp, Listeria grayi
tgccaaaaggtgaaggaaaattaattgcgcaaaataaaaaagccagacatgattttgcaatcgaagaaacttttgaagccggcattgtcttgcaaggaacagagatcaaatccgttcgtaatgcacgagtgaacttaaaggattcttacgcccgcatcgaacgcggagaaatttttttacacaacatgcatatcagcccttacgaccaagggaatagattcaatcatgacccacttcgaactcgtaaattgttattgcacaaaaaacaaatcagccgtctgattggcgaaacaaaagaagctggctattcgatcgtccccctaaagctctatatcaaagatggatttgcaaaagtcttgatcggtgtagctaaagggaagaaaaaatatgacaaacgcgaagatttgaaacgcaaagaagcaaaacgtgatattgaacgagcgtttaaagaaagacaacgataa

SEQ ID NO: 120 - DNA, 465 bp, Listeria monocytogenes
atgccaaaaggtgatggtaagctagtcgcgcaaaataaaaaagcgcgccacgattacgcaattgaagaaacttttgaggctggcattgtcctgcaaggtactgaaattaaatccgtaagaaacgcacgggtaaacttaaaagattcctatgcacgtatcgacaaaggggaaattttcttacacaatatgcatattagtccttatgaacaagggaaccgctacaatcatgatccactaagaacgcgcaagttgctcttacataagaagcaaatcagccgtttaattggagaaacgaaagagtccggttattcgattgttccactaaaaatgtatattaaagatggctacgcaaaagtacttatcggtgtagctcgaggtaaaaagaaatacgataaacgccaagacttaaaacaaaaagaagcaaaacgtgatatcgaacgcgcttttaaagagcgccaacaataa

SEQ ID NO: 121 - DNA, 465 bp, Listeria monocytogenes
atgccaaaaggtgatggtaagctagtcgcgcaaaataaaaaagcgcgccacgattacgcaattgaagaaacttttgaggctggcattgtcctgcaaggtactgaaattaaatccgtaagaaatgcacgggtaaacttaaaagattcctatgcacgtatcgacaaaggggaaattttcttacacaatatgcatattagtccttatgaacaagggaaccgctacaatcatgatccactaagaacgcgcaagttgctcttacataagaagcaaatcagccgtttaattggagaaacgaaagagtccggttattcgattgttccactaaaaatgtatattaaagatggctacgcaaaagtacttatcggtgtagctcgaggtaaaaagaaatacgataaacgccaagacttaaaacaaaaagaagcaaaacgtgatatcgaacgcgcttttaaagagcgccaacaataa

SEQ ID NO: 122 - DNA, 465 bp, Listeria monocytogenes; identical to SEQ ID NO: 121

SEQ ID NO: 123 - DNA, 465 bp, Listeria innocua
atgccaaaaggtgatggtaaactagtcgcgcaaaataaaaaagcgcgccacgattacgcaattgaagaaacttttgaggctggcattgtcctgcaaggtactgaaatcaaatccgtcagaaacgcacgggtaaacttaaaagattcctatgcacgtatcgacaaaggggaaattttcttacacaatatgcacattagtccatatgaacaagggaaccgctacaatcatgatccactaagaacgcgcaagttgctcttacataagaagcaaatcagccgtttaattggagaaacgaaagagtccggttattcgattgttccactaaaaatgtatattaaagatggctacgcaaaagtactcatcggtgtagctcgaggtaaaaagaaatacgataaacgccaagacttaaaacaaaaagaagcaaaacgtgatattgaacgcgcctttaaagagcgccaacaataa

SEQ ID NO: 124 - DNA, 465 bp, Listeria welshimeri
atgccaaaaggtgatggtaaactagtcgcgcaaaataaaaaagcgcgccacgattacgcaattgaagaaacttttgaagctggcattgtcctgcaaggcaccgaaattaaatccgttagaaacgcacgggtaaacttaaaagattcctatgcacgtatcgacaaaggggaaattttcttacacaatatgcatattagcccttatgaacaagggaaccgctacaatcatgatccactaagaacgcgcaaactgcttttacataagaagcaaatcagccgtttaattggcgaaacgaaagaatctggttattcgattgttccgcttaaaatgtatattaaagatggatacgcaaaagtactcatcggtgtagctagaggtaaaaagaaatacgataaacgccaagatttgaaacaaaaagaagcaaaacgtgatattgaacgtgcatttaaagaacgccaacaataa

SEQ ID NO: 125 - DNA, 464 bp, Listeria ivanovii
atgccaaaaggtgatggtaagctagtcgcgcaaaataaaaaagcgcgccacgattacgcaattgaagaaacttttgaggctggcattgtcctgcaaggtactgaaattaaatccgttagaaatgcacgggtaaacttaaaagattcctatgcacgtattgataaaggggaaatttttttacacaatatgcacattagcccatacgaacaagggaaccgctacaaccacgacccactacgaacgcgcaagttgctacttcataaaaaacaaattagccgtttaattggagaaacaaaagagtctggttattcgattgttccgctaaaaatgtatattaaagatggctacgcaaaagtcttaattggagtagctagaggtaaaaagaaatacgataagcgtcaagatttaaaacaaaaagaagcaaaacgtgatattgagcgtgctttcaaagaacgccaacaata

SEQ ID NO: 126 - DNA, 465 bp, Listeria seeligeri
atgccaaaaggtgatggtaagctagtcgcgcaaaataaaaaagcgcgccacgattacgcaattgaagaaacttttgaggctggcattgtcctgcaaggtactgaaattaaatccgttagaaatgcacgggtaaacttaaaagattcctatgcacgtattgataaaggggaaattttcttacacaatatgcacattagcccatacgaacaaggaaaccgttacaatcacgacccactaagaacacgcaaattacttcttcataaaaaacaaatcagtcgtttaattggagaaacaaaagagtccggttattccatcgtcccgctaaaaatgtatattaaagatggttacgcaaaagtattgatcggtgtagctagaggtaaaaagaaatatgataaacgccaagacttaaaacaaaaagaagcaaaacgtgatattgagcgtgctttcaaagaacgccaacaataa

SEQ ID NO: 127 - DNA, 441 bp, Mycoplasma pneumoniae
atgcgagtacttgtcaacaatcccagagcgcaatatgactattaccttttaacgggttattgtgctggcttagtcttaaaaggtagtgaagtcaaatcgctagctttagggcaaggtagcttaaaggaagcctatgtttttattgacaagcacgaggtctatattaaagattttagcatttcgccctatgccttttcaggcgagttcaaccaccccttcaaacgggtgaaaaagctccttttaaaccggaatgagattaaacaaattacggcacgccaaaagcaagaaggactttccattattccacttaaagtgttctttaaaaatggcaaaattaaaatggaaatctggttggccaaacctaagaaaaaatttgataaacgtgaagccatcaaaagtaaaacgatccagcgcgaattgcgccaacaatatggatcgcca

SEQ ID NO: 128 - DNA, 441 bp, Mycoplasma pneumoniae; identical to SEQ ID NO: 127

SEQ ID NO: 129 - DNA, 441 bp, Mycoplasma pneumoniae; identical to SEQ ID NO: 127

SEQ ID NO: 130 - DNA, 441 bp, Mycoplasma pneumoniae; identical to SEQ ID NO: 127

SEQ ID NO: 131 - DNA, 442 bp, Mycoplasma pneumoniae
atgcgagtacttgtcaacaatcccagagcgcaatatgactattaccttttaacgggttattgtgctggcttagtcttaaaaggtagtgaagtcaaatcgctagctttagggcaaggtagcttaaaggaagcctatgtttttattgacaagcacgaggtctatattaaagattttagcatttcgccctatgccttttcaggcgagttcaaccaccccttcaaacgggtgaaaaagctccttttaaaccggaatgagattaaacaaattacggcacgccaaaagcaagaaggactttccattattccacttaaagtgttctttaaaaaatggcaaaattaaaatggaaatctggttggccaaacctaagaaaaaatttgataaacgtgaagccatcaaaagtaaaacgatccagcgcgaattgcgccaacaatatggatcgcca

SEQ ID NO: 132 - DNA, 483 bp, Mycobacterium tuberculosis
gtgtccaagtcgtcgcgtggcggccggcagatcgttgccagcaatcgcaaagcccggcacaactattcgatcatcgaggtgttcgaggccggggttgcgctgcaaggcacggaggtgaagagcctgcgggaagggcaggcgtcgctggccgattcgttcgccaccatcgacgacggcgaagtgtggctgcgcaacgcgcacatcccggaataccggcacggcagctggaccaaccacgagccgcgacgcaaccgcaaactgctgttgcatcgccgccagatcgacaccttggtcggcaagatccgcgaaggcaacttcgccctggtgccgttgtcgctgtatttcgccgaaggcaaggtcaaggttgagcttgcgctggcccgaggcaagcaagcccgcgacaaacgccaggacatggcccgtcgtgatgcccagcgtgaagtgctccgcgagttgggtcggcgcgctaagggcatgacctga

SEQ ID NO: 133 - DNA, 483 bp, Mycobacterium bovis; identical to SEQ ID NO: 132

SEQ ID NO: 134 - DNA, 483 bp, Mycobacterium bovis; identical to SEQ ID NO: 132

SEQ ID NO: 135 - DNA, 483 bp, Mycobacterium canettii; identical to SEQ ID NO: 132

SEQ ID NO: 136 - DNA, 483 bp, Mycobacterium africanum; identical to SEQ ID NO: 132

SEQ ID NO: 137 - DNA, 483 bp, Mycobacterium lepraestrain
gtggccagaaaccctcgtggcggcaagcagattgtggccaccaatcgcaaggctcggcacgattacgcaatcattgaattgtttgaggctggggtggcgttgcttggcaccgaggtgaaaagtctgcgggaggggcatgcgtcgctggccgacgcgttcgcaaccgtcgacagcggtgaagtgtggttgcgaaacatgcacatcccggagtatcagcatggtagctggaccaatcacgatcctcgccgtaaccgcaagctgctgctgcaccgccgccagatcgacaccctggttggcaagatccgtgacggcaacctcgcgctagtgccgttatcgttgtattttgccgagggcaaggtcaaggtcgagcttgcgctggcgcgcggcaagaaactgcacgacaagcgccaggacatggcgcgtcgcgatgctcagcgcgaagtaatccgtgaactcggtcgccgtgccaagggcatgctctga

SEQ ID NO: 138 - DNA, 486 bp, Mycobacterium smegmatis
gtgaccaagaagagcgcctccagcaacaacaaggtggtcgccaccaaccgcaaggcgcgacacaactacacgatcctcgacacctacgaggccgggatcgtgttgatgggcacggaggtcaagagcctgcgcgaaggtcaggcctcgctggccgacgcgttcgccacggtcgacgacggcgagatctggctgcgcaacgtccacatcgccgaatatcaccacggcacctggaccaaccacgcgccgcggcgcaaccgcaaactgctgctgcaccgcaagcagatcgacaacctcatcggcaagatccgcgacggcaacctcacgctggtgccgctgtcgatctacttcaccgacggcaaggtcaaggtcgagttggcgctcgcccgcggcaagcaggcccacgacaagcgccaggacctcgcccgtcgagacgctcaacgcgaggtgatccgcgagctgggccgccgggccaagggcaagatctga

SEQ ID NO: 139 - DNA, 510 bp, Mycobacterium intracellulare
gtggccaagggatccggccgggccaaggcggcgggcggcaaaggcggcagcaaacaagttgtggccaccaatcgcaaagcgcggcataactattcgatcatcgaatcgttcgaggccggggtcgcgctgcaaggcaccgaggtcaaaagcctgcgcgagggccaagcttcgttagctgacgccttcgcaacgatcgacgacggcgaagtgtggttgcgcaacttgtacattgcggagtaccagcacggtagctggaccaatcatgacccccggcgcaaccgaaagttgttgttacatcggcaacaaatcgacaggctggtcggcaagattcgagatggtaacctcgccttgatgccgctgtctctgtatttctccgagggcaaggtcaaggtcgaactggcccttgcgcgcggcaaaagggcttacgacaaacgccaggacatggcccagcgcgacgcacagcgcgaagtggtccgtgaactagggcgccgagcgaagggcatgacctga

SEQ ID NO: 140 - DNA, 510 bp, Mycobacterium avium
gtggccaagggttccggccgggccaaagcggcgggcggcaaaggtggcagcaaacagatcattgccaccaatcgcaaagcgcggcacaactattcgatcatcgaaacgtacgaggccggggtggcgttgcaaggaaccgaggtcaaaagcctgcgggagggccaagcgtcgttagctgacgcgttcgcaacgatcgacgacggtgaagtctggttgcgcaacttgtacatcccggagtatcaacacggtagctggaccaatcacgacccacgccggaaccgaaagttgttgttacataggcaacaaatcgacagactggtcggcaagatccgggatggtaacctcgccttgatgccgctgtcgctgtacttctccgagggcaaagtgaaggtagagctcgctctcgcgcgcggcaagaaggcttacgacaaacgccaggacctggcccagcgcgacgcacagcgcgaagtcgttcgtcaactgggacgccgaacaaaggggatgatctga

SEQ ID NO: 141 - DNA, 510 bp, Mycobacterium avium; identical to SEQ ID NO: 140

SEQ ID NO: 142 - DNA, 480 bp, Mycobacterium abscessus
atgagtaagaaaccggccgacggacgaaaagtcatcgcgaccaatcgcaaggcacgacacaactattcgatcatcgatgtgtatgaggccggggtgcagttggtgggcaccgaggtcaagacactgcgcgagggcaaggcatcgctggtcgatgccttcgccaccgtcgatgacggcgaggtgtggttgcgcggcgtgcatatcccgcaatacgaccacggcacctggaccaatcacgctccgctgcggaaccggaaactgttgttgcacagggcgcagatcgacatgctggtcggcaagacccgcgacggcaatctgaccctggtaccgctgtcgctgtacttcctggacggcaaggtcaaggtggagttggcgctggcgcggggtaagcaggctcacgacaagcgtcaggacatcgccaaacgggacgcttcgcgtgagatcacccgtgagctgggacgccgcgccaaaggcatgtga

SEQ ID NO: 143 - DNA, 406 bp, Legionella pneumophila
gggggcgacctggcttcgacgtgggttgcaaaaccggaagtgcatgccgagaaggagatctctcgtaaataagactcaattaaatataaatgcaaacgatgaaaactttgctggtggggaagctatcgctgcctaataagcactttagttaaaccatcactgtgtactggccaataaacccagtatcccgttcgaccgagcccgcttatcggtatcgaatcaacggtcataagagataagctagcgtcctaatctatcccgggttatggcgcgaaactcagggaatcgctgtgtatcatcctgcccgtcggaggagccacagttaaattcaaaagacaaggctatgcatgtagagctaaaggcagaggacttgcggacgcgggttcgattcccgccgcctccacca

SEQ ID NO: 144 - DNA, 406 bp, Legionella pneumophila; identical to SEQ ID NO: 143

SEQ ID NO: 145 - DNA, 406 bp, Legionella pneumophila; identical to SEQ ID NO: 143

SEQ ID NO: 146 - DNA, 406 bp, Legionella pneumophila; identical to SEQ ID NO: 143

SEQ ID NO: 147 - DNA, 406 bp, Legionella pneumophila; identical to SEQ ID NO: 143

SEQ ID NO: 148 - DNA, 406 bp, Legionella pneumophila; identical to SEQ ID NO: 143

SEQ ID NO: 149 - DNA, 406 bp, Legionella pneumophila
gggggcgacctggcttcgacgtgggttgcaaaaccggaagtgcatgccgagaaggagatctctcgtaaataagactcaattaaatataaatgcaaacgatgaaaactttgctggtggggaagctatcgctgcctaataagcactttagttaaaccatcactgtgtactggccaataaacccagtatcccgttcgaccgagcccgcttatcggtatcgaatcaacggtcataagagataagctagcgtcctaatctatcccgggttatggcgcgaaattcagggaatcgctgtgtatcatcctgcccgtcggaggagccacagttaaattcaaaagacaaggctatgcatgtagagctaaaggcagaggacttgcggacgcgggttcgattcccgccgcctccacca

SEQ ID NO: 150 - DNA, 406 bp, Legionella pneumophila; identical to SEQ ID NO: 149

SEQ ID NO: 151 - DNA, 406 bp, Legionella pneumophila
gggggcgacctggcttcgacgtgggttgcaaaaccggaagtgcatgccgagaaggagatctctcgtaaataagactcaattaaatataaatgcaaacgatgaaaactttgctggtggggaagctatcgctgcctaataagcactttagttaaaccatcactgtgtactggccaataaacccagtatcccgttcgaccgagcccgcttatcggtatcgaatcaacggtcataagagataagctagtgtcctaatctatcccgggttatggcgcaaaactaagggaatcgctgtgtatcatcctgcctgtcggaggagccacagttaaattcaaaagacaaggctatgcatgtagagctaaaggcagaggacttgcggacgcgggttcgattcccgccgcctccacca

SEQ ID NO: 152 - DNA, 405 bp, Legionella longbeachae
gggggcgacctggcttcgacgtgggttgcaaaaccagaggtgcatgccgagaatgaggactctcgtaaatcagactcaactaaatataaatgcaaacgatgaaaactttgctggtggggaagctattgctgcctaataagcactttagataaaccatcactgtgtactggccaataaacccagtatcccgttcgaccgagcccgcttatcggtatcgaatcaacggtcataagagataagctagcgtcctaatccatcccgtattaaggcgcgaaactcagggaatcgctgtgtagtatcctgcccgtcggagaatgcacagttaaatcaaaagacaaggctacgcatgtagagctgaaggcagaggatttgcggacgcgggttcgattcccgccgcctccacca

SEQ ID NO: 153 - DNA, 405 bp, Legionella longbeachae; identical to SEQ ID NO: 152

SEQ ID NO: 154 - DNA, 414 bp, Legionella fallonii
gggggcgacctggcttcgacgtgggttgcaaaaccggaagtgcatgccgagaatgagaactctcgtaaatcagactcactaaatataaatgcaaacgaagaaaacttcgatggcgtagctaatcttgaaggagtagcgcaagctgcttaatcttttttagttaaaccataacgtgtactggctttaaccccagtgccccgttgaccgagctcgcttatcggtatcgaatcaacggtcatagaagataagctagtgtcctaatctatcccgggttacgatgcgaaactcagggagtagctgtgtaccatcctgcctgtcggagagtccacagttaaatcaaatgacaaggctacgcatgtagagctgaaggcagaggatttgcggacgcgggttcgattcccgccgcctccacca

SEQ ID NO: 155 - DNA, 395 bp, Legionella hackeliae
gggggcgacctggcttcgacgtgggttgcgaaacctgaagtgcatgccgagaatgagacgtctcgtaaatcagactcactaaatataaatgcaaacgatgaaaactttgcaggtgaagctatcgctgcgtaagctttgatagtgtaaccgcaccgtgcgctgctatataaccagcgccccgttgaccgagctcgcttatcggtatcgaatcaacggtcatagaagataagctcgcatcttaacccgtcccgagttaagctgttaaattaagggaatcgccgtgttcaatcctgcccgtcggagggaccacggttaacttaaaagacaaggctacgcatgtagagctgatggcagaggatttgcggacgcgggttcgattcccgccgcctccacca

SEQ ID NO: 156 - DNA, 410 bp, Legionella oakridgensis
gggggcgacctggcttcgacgtgggttgcgaaacctgaagtgcatgccgagaatgagatctctcgtaaataaggctcactaaatataaatgcaaatgatgaaaactttgctggtgttgagggagaagctatcgctgcgtaagcattgatggttttaccaaaaacatcactgtgcgctgccaaaaaccagcgccccgttgaccgagctcgcttgtcggtatcgaatcaacggtcatagaagataagctagtcttttgatttgtcccgcatcaaagggcgaaattcagggaatcgccgtgtatcatcctgccagtcggagggtccacggtcagaataatagaccaggctaagcatgtagagctgatggcagaggatttgcggacgcgggttcgattcccgccgcctccacca

SEQ ID NO: 157 - DNA, 404 bp, Legionella micdadei
gggggcgacctggcttcgacgtgggttgcgaaacctgaggtgcatgccgagaatgagatctctcgtaaataagactcactaaatataaatgcaaacgatgaaaactttgctggtggagaaggcgctatcgctgcgtaagcattgatagaaacttttccccaatcgtgcgctgccaaaaaccagcgccccgttgaccgagctcgcttaccggtatcgaatcaacggtcataagagataagctcgcaacttggttagtcccgcatcaagttgttaaatccagggaatcgccgtaaaccatcctgcctgtcggaggggctacggttaacttaatagacaaggctaagcatgtagaactgatggcagaggatttgcggacgcgggttcaattcccgccgcctccacca

SEQ ID NO: 158 - DNA, 405 bp, Legionella sainthelensi
gggggcgacctggcttcgacgtgggttgcaaaaccagaggtgcatgccgagaatgaggactctcgtaaatcagactcaactaaatataaatgcaaacgatgaaaactttgctggtggggaagctattgctgcctaataagcactttagttaaaccatcactgtgtactggccaataaacccagtatcccgttcgaccgagcccgcttatcggtatcgaatcaacggtcataagagataagctagcgtcctaatccatcccgtattaaggcgcgaaacttagggaatcgctgtgtagtatcctgcccgtcggagaatgcacagttaaatcaaaagacacggctacgcatgtagagctgaaggcagaggatttgcggacgcgggttcgattcccgccgcctccacca

SEQ ID NO: 159 - DNA, 406 bp, Legionella wadsworthii
gggggcgacctggtttcgacgtgggttgcaaaaccagaggtgcatgccgagattgagaactctcgtaaatcagactcaacttaaatataaatgcaaacgatgaaaactttgctggtggagaagctatcgctgcctaataagcactttagttgaaccatcactgtgtactggccaataaacccagtatcccgttcgaccgagcccgcttatcggtatcgaatcaacggtcataagagataagctagcgtcctaatccatcccgtattaaggcgcgaaattcagggaatcgctgtgtagtatcctgcccgtcggagaatgcacagttaaatcaaaagacacggctacgcatgtagagctgaaggcagaggacttgcggacgcgggttcgattcccgccgcctccacca

SEQ ID NO: 160 - DNA, 405 bp, Legionella cherrii
gggggcgacctggcttcgacgtgggttgcaaaaccagaggtgcatgccgagaatgagaactctcgtaaatcagactcaactaaatataaatgcaaacgatgaaaactttgctggtggggaagctatcgctgcctaataagcactttagttaaaccatcactgtgtactggccaataaacccagtatcccgttcgaccgagcccgcttatcggtatcgaatcaacggtcataagagataagctagtgtcttaatccatcccgtattaagatgcgaaattcagggaatcgctgtgtagtatcctgcccgtcggagaatgcacagttaaatcaaaagacacggctacgcatgtagagctgaaggcagaggatttgcggacgcgggttcgattcccgccgcctccacca

SEQ ID NO: 161 - DNA, 405 bp, Legionella moravica
gggggcgacctggcttcgacgtgggttgcaaaaccagaggtgcatgccgagaatgagaactctcgtaaatcagactcaactaaatataaacgcaaacgatgaaaactttgctggtggagaagctatcgctgcctaataagcactttagttgaaccatcactgtgtactggccaataaacccagtatcccgttcgaccgagcccgcttatcggtatcgaatcaacggtcataagagataagctagtgtcttaatccatcccgaattaaggcgcgaaattcagggaatcgctgtgtagtatcctgcctgtcggagaatgcacagttaaattaaaagacaaggctacgcatgtagagctgaaggcagaggatttgcggacgcgggttcgattcccgccgcctccacca

SEQ ID NO: 162 - DNA, 404 bp, Legionella norrlandica
gggggcgacctggcttcgacgtgggttgcaaaaccggaagtgcatgccgagaatgagatctctcgtaaataagactcaattaaatataaatgcaaacgatgaaaactttgctggtggtgaagctatcgctgcctaataagcacgattagataaaccccaatcgtgtactggccaaaaacccagtatcccgttgaccgagctcgcttatcggtatcgaatcaacggtcatagaagataagctagtactttaatctatcctgggttatggtgcgaaatttagggaatcgctgtgtatcatcctgcccgtcggaggagccacagttaaatttaatagacaaggctaagcatgtagagctaaaggcagaggacttgcggacgcggttcgattcccgccgcctccacca

SEQ ID NO: 163 - DNA, 401 bp, Legionella shakespearei
gggggcgacctggcttcgacgtgggttgcgaaaccggaagtgcatgccgagaatgagaactctcgtaaatcagactcaaaaaatataaatgcaaacgatgcaaacttcgctgataacgttgatggagcaattgctgcttaatcaatagttaaaagcaacgtgtactggcctaaaccccggtgccccgttgaccgagctcgcttattggtatcgaatcaacggtcatagaagataagctagcttcttaatgaatcccgagttaagacgcgaaattcagggaatcgctgtgtaccatcctgcccgtcggagtgtccacagttaaaccaaaagacaaggctacgcatgtagagctaaaggcagaggatttgcggacgcgggttcgattcccgccgcctccacca

SEQ ID NO: 164 - DNA, 405 bp, Legionella drancourtii
gggggcgacctggcttcgacgggggttgcaaaaccagaggtgcatgccgagaatgagatctctcgtaaatcaggctcaataaatataaatgcaaacaatgcaaactttgatgatgtttcttttgacggggctattgcagcttaatcagattaaactaatcgacgtgtactggccttaaccccagtgccccgttgaccgagctcgcttattggtatcgaatcaacggtcatagaagataagctagtgttttaatttatcccggattaaaatgcgaaactcagggaatcgctgtgtaccatcctgcctgtcggagagtccacagttaaatcaaatgacaaggctacgcatgtagaactgaaggcagaggatctgcggacgcgggttcgattcccgccgcctccacca

SEQ ID NO: 165 - DNA, 399 bp, Legionella lansingensis
gggggcgacctggcttcgacgtgggttgcgaaacctgatgtgcatgccgagaaagagtactctcgtaaatcagtctcactaaatataaatgcaaacgatgaaaactttgctggtggtgaagctgtcgctgcgtaagctttgatagtcaactaccgatagtgcgctgccataaaaccagcgccccgttgaccgagctcgcttatcggtatcgaatcaacggtcataagagataagctcgcatcttggttcgtcccgcaccaagatgttaaatcaagggaatcgccgtgtcccatcctgcctgtcggagaggccacggttaactaaaaagacaaggctaagcatgtagatctgacggcagaggatttgcggacgcgggttcgattcccgccgcctccacca

SEQ ID NO: 166 - DNA, 396 bp, Legionella fairfieldensis
gggggcgacctggcttcgacgcgggttgcgaaacctgaggggcatgccgagaatgagaactctcgtaaatcagactcactaaatataaatgcaaacgatgaaaactttgcaggtgaagctatcgctgcttaagctttgatagtttaaccgcaccgtgcgctgccataaaaccagcgccccgttgaccgagcttgcttatcggtatcgaatcaacggtcatagaagataagctcgcattttggtacgtcccgcatcaaaatgttaaattaagggaatcgccgtgtactatcctgcctgtcggagagtccacggttaacataaatagacaaggctacgcatgtagaactgacggcagaggatttgcggacgcgggttcgattcccgccgcctccacca

SEQ ID NO: 167 - DNA, 401 bp, Legionella massiliensis
gggggcgacctggcttcgacgtgggttgcgaaacctgatgtgcatgccgagattgagacttctcgttaatcagactcactaaacataaatgcaaacgatgaaaactttgcagatggagaagctatcgctgcgtaagctttgataggtttttcgtcgcaccgtgtgctgctataaaaccagcaccccgttgaccgagcttgcttatcggtatcgaatcaacggtcatagaagataagctcgcagcttgatatttcccgtatcaagatgttaaatccagggaatcgccgcgaaccatcctgcctgtcggaggggactcggttaattgaatagacaaggctacgcatgtagagctgacggcagaggatttgcggacgcgggttcaattcccgccgcctccacca

SEQ ID NO: 168 - DNA, 396 bp, Legionella geestiana
gggggcgacctggcttcgacgtgggttgcgaaacctgatgtgcatgccgaggatgagaactctcgtaaaacgggctcgataaatataaatgcaaacgatgaaatgttcgctggagaagctgtagctgcgtaagcaactgcggtgaccgaagcacagtgcgctgccaaaaacccagcgccccgttgaccgggcttgcttgccggtaccgaatcaacggtcatagaagacaagctggtatcctggtgtatcccgcgccagtatacaagactcagggaatcgctgccgaccatcctgcctgtcggaggggaagcagttaaaacaaatgacaaggctaagcatgtagatctgacggcagaggatttgcggacgcgggttcgattcccgccgcctccacca

SEQ ID NO: 169 - DNA, 486 bp, Haemophilus influenzae; identical to SEQ ID NO: 1

SEQ ID NO: 170 - DNA, 486 bp, Haemophilus influenzae
atgacaaagaaaaaagtaaaacccaattcaaatactatcgcactaaataaacgtgcaagacacgattattttattgaagatgaaattgaagcaggtcttgaattacaaggctgggaagtcaaatctatgcgcgcaggcaaggcaaatattagtgatagttatgttatttttaaaaatggcgaagcctttttattcggcgcaagcattcagccattaaatgttgcatcaacgcatattgtttgtgatccaactcgcactcgtaagttattgttaaataaacgcgaattagcatccctatttggtaaagcaaaccgagacggttttaccatagttgcactttctctttactggaaaagtgcgtgggcaaaagtcaaaatcggtttagccaaaggtaaaaaacaacaggataaacgtgatgatattaaagaacgtgaatggaaagtaacaaaagatcgcattatgaaaaatgcacatcgaagatcttaa

SEQ ID NO: 171 - DNA, 486 bp, Haemophilus influenzae
atgacaaagaaaaaagtaaaacccaattcaaatactatcgcactgaataaacgtgcaagacacgattattttattgaagatgaaattgaagcaggtcttgaattacaaggctgggaagtcaaatctatgcgcgcaggcaaggcaaatattagtgatagttatgttatttttaaaaatggcgaagcctttttattcggcgcaagcattcagccattaaatgttgcatcaacgcatattgtttgtgatccaactcgcactcgtaagttattgttaaataaacgcgaattagcatccctatttggcaaagcaaaccgagacggttttaccatagttgcactttctctttactggaaaagtgcgtgggcaaaagtcaaaatcggtttagccaaaggtaaaaaacaacaggataaacgtgatgatattaaagaacgtgaatggaaagtaacaaaagatcgcattatgaaaaatgcacatcgaagatcttaa

SEQ ID NO: 172 - DNA, 486 bp, Haemophilus influenzae
atgacaaagaaaaaagtaaaacccaattcaaatactatcgcactgaataaacgtgcaagacacgattattttattgaagatgaaattgaagcaggtcttgaattacaaggctgggaagtcaaatctatgcgcgcaggcaaggcaaatattagtgatagttatgttatttttaaaaatggcgaagcctttttattcggcgcaagcattcagccattaaatgttgcatcaacgcatattgtttgtgatccaactcgcactcgtaagttattgttaaataaacgcgaattagcatccctatttggcaaagcaaaccgagacggttttaccatagttgcactttctctttactggaaaagtgcgtgggcaaaagtcaaaattggtttagccaaaggtaaaaaacaacaggataaacgtgatgatattaaagaacgtgaatggaaagtaacaaaagatcgcattatgaaaaatgcacatcgaagatcttaa

SEQ ID NO: 173 - DNA, 486 bp, Haemophilus influenzae
atgacaaagaaaaaagtaaaacccaattcaaatactatcgcactaaataaacgtgcaagacacgattattttattgaagatgaaattgaatcaggtcttgaattacaaggctgggaagtcaaatctatgcgcgcaggcaaggcaaatattagtgatagttatgttatttttaaaaatggcgaagcctttttattcggcgcaagcattcagccattaaatgttgcatcaacgcatattgtttgtgatccaactcgcactcgtaagttattgttaaataaacgcgaattagcatccctatttggcaaagcaaaccgagacggttttaccatagttgcactttctctttactggaaaagtgcgtgggcaaaagtcaaaattggtttagccaaaggtaaaaaacaacaggataaacgtgatgatattaaagaacgtgaatggaaagtaacaaaagatcgcattatgaaaaatgcacatcgaagatcttaa

SEQ ID NO: 174 - DNA, 486 bp, Haemophilus influenzae
atgacaaagaaaaaagtaaaacccaattcaaatactatcgcactgaataaacgtgcaagacacgattattttattgaagatgaaattgaagccggtcttgaattacaaggctgggaagtcaaatctatgcgcgcaggcaaggcaaatattagtgatagttatgttatttttaaaaatggcgaagcctttttattcggcgcaagcattcagccattaaatgttgcatcaacgcatattgtttgtgatccaactcgcactcgtaagttattgttaaataaacgcgaattagcatccctatttggcaaagcaaaccgagacggttttaccatagttgcactttctctttactggaaaagtgcgtgggcaaaagtcaaaatcggtttagccaaaggtaaaaaacagcaggataaacgtgatgatattaaagaacgtgaatggaaagtaacaaaagatcgcattatgaaaaatgcacatcgaagatcttaa

SEQ ID NO: 175 - DNA, 486 bp, Haemophilus influenzae
atgacaaagaaaaaagtaaaacccaattcaaatactatcgcactgaataaacgtgcaagacacgattattttattgaagatgaaattgaagcaggtcttgaattacaaggctgggaagtcaaatctatacgcgcaggcaaggcaaatattagtgatagttatgttatttttaaaaatggcgaagcctttttattcggcgcaagcattcagccattaaatgttgcatcaacgcatattgtttgtgatccaactcgcactcgtaagttattgttaaataaacgcgaattagcatccctatttggcaaagcaaaccgagacggttttaccatagttgcactttctctttactggaaaagtgcgtgggcaaaagtcaaaattggtttagccaaaggtaaaaaacaacaggataaacgtgatgatattaaagaacgtgaatggaaagtaacaaaagatcgcattatgaaaaatgcacatcgaagatcttaa

SEQ ID NO: 176 - DNA, 486 bp, Haemophilus influenzae
atgacaaagaaaaaagtaaaacccaattcaaatactatcgcactgaataaacgtgcaagacacgattattttattgaagatgaaattgaagcaggtcttgaattacaaggctgggaagttaaatctatgcgcgcaggcaaggcaaatattagtgatagttatgttatttttaaaaatggcgaagcctttttattcggtgcaagcattcagccattaaatgttgcatcaacgcatattgtttgtgatccaactcgcactcgtaagttattgttaaataaacgcgaattagcatccctatttggcaaagcaaaccgagacggttttaccatagttgcactttctctttactggaaaagtgcgtgggcaaaagtcaaaattggtttagccaaaggtaaaaaacaacaggataaacgtgatgatattaaagaacgtgaatggaaagtaacaaaagatcgcattatgaaaaatgcacatcgaagatcttaa

SEQ ID NO: 177 - DNA, 486 bp, Haemophilus influenzae; identical to SEQ ID NO: 176

SEQ ID NO: 178 - DNA, 486 bp, Haemophilus influenzae
atgacaaagaaaaaagtaaaacccaattcaaatactatcgcactgaataaacgtgcaagacacgattattttattgaagatgaaattgaagcaggtcttgaattacaaggctgggaagtcaaatctatgcgcgcaggcaaggcaaatattagtgatagttatgttatttttaaaaatggcgaagcctttttattcggggcaagcattcagccattaaatgtcgcatcaacgcatattgtttgtgatccaactcgcactcgtaagttattgttaaataaacgcgaattaacatccctatttggcaaagcaaaccgagacggttttaccatagttgcactttctctttactggaaaagtgcgtgggcaaaagtcaaaattggtttagccaaaggtaaaaaacaacaggataaacgtgatgatattaaagaacgtgaatggaaagtaacaaaagatcgcattatgaaaaatgcacatcgaagatcttaa

SEQ ID NO: 179 - DNA, 481 bp, Haemophilus haemolyticus
atgacaaagaaaaaagtaaaaccaggatcaaacactatcgcactgaataaacgtgcgagacatgattattttatagaagatgaaattgaagcgggtcttgaattacaaggctgggaagtcaaatcaatgcgcgcaggcaaggcaaacattagtgatagttatgtcatttttaaaaatggcgaagcctttttattcggcgcaagcattcagccattaaatgttgcatcaacgcatattatttgtgatccaactcgcactcgtaagttattattaaataaacgcgaattagcatccctatttggcaaagcaaaccgagacggttttaccatcgtagcgctttctctttattggaaaagtgcatgggcaaaagtcaagattggtttagccaaaggtaaaaaacaacatgataaacgcgatgatattaaagagcgtgaatggaaagtaacaaaagatcgcattatgaaaaatgcacatcgaggat

SEQ ID NO: 180 - DNA, 481 bp, Haemophilus haemolyticus
atgacaaagaaaaaagtaaaaccaggatcaaatactatcgcactgaataaacgtgcgaaacatgattattttatagaagatgaaattgaagcaggtcttgaactacaaggctgggaagtcaaatcaatgcgcgcaggcaaggcaaacattagtgatagttatgtcattttcaaaaatggcgaagcctttttattcggtgcaagcattcagccattaaatgttgcatcaacgcatattgtttgtgatccaactcgcactcgtaagttattattaaataaacgcgaattagcatccctatttggcaaagcaaaccgagacggttttaccatcgtagcgctttctctttattggaaaagtgcatgggcaaaagtcaaaattggtttagccaaaggtaaaaaacaacatgataaacgcgatgatattaaagagcgtgaatggaaagtaacaaaagatcgcattatgaaaaatgcacatcgaggat

SEQ ID NO: 181 - DNA, 481 bp, Haemophilus haemolyticus
atgacaaagaaaaaagtaaaaccagaatcaaatactattgcactgaataaacgtgctagacatgactattttatagaagatgaaattgaagcgggtcttgaattacaaggctgggaagtcaaagcaatgcgcgcaggcaaggcaaacattagtgatagttatgtcatttttaaaaatggcgaagcctttttattcggggcaagcattcagccattaaatgttgcatcaacgcatattgtttgtgatccaactcgcactcgtaagttattattaaataaacgcgaattagcatccctatttggcaaagcaaaccgagacggttttaccatcgtagcgctttctctttattggaaaagtgcatgggcaaaagtcaaaattggtttagccaaaggtaaaaaacaacatgataaacgcgatgatattaaagagcgtgaatggaaagtaacaaaagatcgcattatgaaaaatgcacatcgaggat

SEQ ID NO: 182 - DNA, 481 bp, Haemophilus haemolyticus
atgacaaagaaaaaagtaaaaccaggatcaaacactatcgcactgaataaacgtgcgagacatgattattttatagaagatgaaattgaagcgggtcttgaattacaaggctgggaagtcaaatcaatgcgcgcaggcaaggcaaacattagtgatagttatgtcatttttaaaaatggcgaagcctttttattcggggcaagcattcagccattaaatgttgcatcaacacatattgtttgtgatccaactcgcactcgtaagttattattaaataaacgcgaattagcatccctatttggcaaagcaaaccgagacggttttaccatcgtagcgctttctctttattggaaaagtgcatgggcaaaagtcaaaattggtttagccaaaggtaaaaaacaacatgataaacgcgatgatattaaagagcgtgaatggaaagtaacaaaagatcgcattatgaaaaatgcacatcgaggat

SEQ ID NO: 183 - DNA, 481 bp, Haemophilus haemolyticus
atgacaaagaaaaaagtaaaaccaggatcaaatactatcgcactgaataaacgtgcgagacatgattattttatagaagatgaaattgaagcaggtcttgaactacaaggctgggaagttaaatcaatgcgcgcaggcaaggcaaacattagtgatagttatgtcatttttaaaaatggcgaagcctttttattcggtgcaagcattcagccattaaatgtagcatcaacgcatattgtttgtgatccaactcgcactcgtaagttattattaaataaacgtgaattagaatccctatttggcaaagcaaaccgagacggttttaccatcgtagcgctttctctttactggaaaagtgcatgggcaaaagtcaaaattggtttagccaaaggtaaaaaacaacatgataaacgcgatgatattaaagagcgtgaatggaaagtaacaaaagatcgcattatgaaaaattcacatcgaggat

SEQ ID NO: 184 - DNA, 480 bp, Haemophilus haemolyticus
atgacaaagaaaaagtaaaaccaggatcaaatactatcgcactgaataaacgtgcgagacatgattattttatagaagatgaaattgaagcaggtcttgaactacaaggctgggaagtcaaatcaatgcgcgcaggcaaggcaaacattagtgatagttatgtcattttcaaaaatggcgaagcctttttattcggcgcaagcattcagccattaaatgttgcatcaacgcacattgtttgtgatccaactcgcactcgtaagttattattaaataaacgtgaactagcatccctatttggcaaagcaaaccgagacggttttaccatcgtagcgctttctctttactggaaaagtgcatgggcaaaagtcaaaattggtttagctaaaggtaaaaaacaacatgataaacgcgatgatatcaaagagcgtgaatggaaagtaacaaaagatcgcattatgaaaaatgcacatcgaggat

SEQ ID NO: 185 - DNA, 483 bp, Haemophilus parainfluenzae
atgaccaagaaaaaagtcaaagtcggctccagcaccattgcgttaaataaacgagccagacacgaatattttattgaagatgaaattgaagccggccttgaattacaaggttgggaagtgaaatcaatgcgcgcgggtaaagccaatatcagcgacagctatatcatttttaaaaacggtgaagcttatttatttggtgcaaccattcaaccattaagcttggcttctacccacgtggtttgcgatccgactcgcacacgtaagcttttattgaataaacgtgaactggataatcttttcggtaaatcaagccgtgatggttttaccattgttgccctttctctttattggaaaggtccttgggcaaagatcaaaatcggtcttgcgaaaggtaaaaaacaacatgataaacgtgatgatattaaagagcgtgaatggaaagtggcaaaagagcgtattatgaaaaatgcgcatcgtggataa

SEQ ID NO: 186 - DNA, 476 bp, Haemophilus parainfluenzae
atgaccaagaagaaagtcaaagtcggctccaataccattgcgttaaataaacgagctcgacacgaatattttattgaagatgaaattgaagccggtcttgaattacaaggttgggaagtgaaatcaatgcgcgcaggtaaagccaatatcagcgacagctatatcatttttaaaaacggggaagcctatttatttggtgcgaccattcaaccattaagcttggcttctactcacgtggtttgcgatccgacgcgtacacgtaagcttttattgaataaacgtgaactggataatcttttcggtaaatcaagccgtgatggttttaccattgttgccctttctctttattggaaaggcccttgggcaaagatcaaaatcggccttgcgaaaggtaaaaaacaacatgataaacgtgatgatattaaagagcgtgaatggaaagtggcgaaagagcgtattatgaaaaacgcgcaccg

SEQ ID NO: 187 - DNA, 477 bp, Haemophilus somnus
atgacaaagaaaaaagcaaaggtagcatctaatacgattgccttaaataaacgagcaagacacgattattttattgaagatgaaatcgaagccggtctttctttgcaaggctgggaagttaaatcgatgcgtgcaggtaaagcgagtattggcgatagttatattatttttaagcatggcgaggcatatttatttggtgcaaccattcagccgttaagtgttgcttcaacgcatattgtttgcgatcccacaagaacacgtaaacttttattaaaccagaaagagttggcttcattatttggtaaagcaaatcgagatggtttcactattgttgcactttcattatattggaaaggtccttgggcaaaggtgaaaataggtttagcaaaagggaaaaaattacatgataagcgtgaagatattaaagatcgtgaatggaaagtaacgaaagatcgcattatgaaaaatgcacagcga

SEQ ID NO: 188 - DNA, 477 bp, Haemophilus somnus
atgacaaagaaaaaagcaaaggtagcatctaatacgattgccttaaataaacgagcaagacacgattattttattgaagatgaaatcgaagccggtctttctttgcaaggctgggaagttaaatcgatgcgtgcaggtaaggcgagtattggcgatagttatattatttttaagcatggtgaggcatatttatttggtgcaaccattcagccgttaagtgttgcttcaacgcatattgtttgcgatcccacaagaacacgtaaacttttattaaaccagaaagagttggcttcattatttggtaaagcaaatcgagatggtttcactattgttgcactttcattatattggaaaggtccttgggcaaaggtgaaaataggtttagcaaaagggaaaaaattacatgataagcgtgaagatattaaagatcgtgaatggaaagtaacgaaagatcgcattatgaaaaatgcacagcga

SEQ ID NO: 189 - DNA, 443 bp, Haemophilus ducreyi
tcaaacacgattgcactcaacaaacgagcccgccacgaatattttattgaagatgaaattgaagcaggtttagcattgcaaggctgggaagttaaatctttacgcgcaggtaaagcaaatatcggtgatagctatgttacttttcgtcatggtgaagcctttttatttggcgctacaattaccccattaaatatggcttctactcatattgttgcagatccaacacgtactcgtaagctactattaaatcaaagagaattagactcattatttggtaaagtaaatcgagatggaatgactgtggtggcactttcgctttattggaaaaatgcttgggcgaaagtcaagatagggctagcgaaaggcaaaaaacttcacgataaacgtgaagatattaaagatcgtgaatggcacgttactaagcaacgcattatgaaaaatgc

SEQ ID NO: 190 - DNA, 483 bp, Haemophilus pittmaniae
atgaccaagaaaaaagctaaagttggcgcaaacaccatcgcattaaacaaacgcgcgcgccacgattattttattgaagacgaagttgaagccggtttggagttgcaaggttgggaagtaaaatccatgcgcgctggtaaagctaatatcagcgacagttacattattttcaaaaatggcgaggcttatttatttggcgcgaccattcagcctttatctctagcatccacccatgtggtttgcgatccgacccgcacccgtaaactgttactcaataaacgcgaactggataatctttttggtaaatcagcacgtgatggttttaccatcgtagcgctttccctttattggaaaggcgcctgggcaaaaattaaaatcggtttggcgaagggtaagaaacaacatgacaaacgcgaagacatcaaagaacgcgaatggaagttggataaacaacgaattatgaaaaatgccaatcgcggctaa

SEQ ID NO: 191 - DNA, 480 bp, Haemophilus sputorum
atggcaaaaaaacctaaagttgcttcaaatactattgcgctaaataaacgcgcacgacatgaatattttattgaagaagaaattgaagccggcttagaactccaaggttgggaagtgaaatctctgcgcgccggtaaagctaatattggggatagctatgttacctttagaaacggcgaagcctttttattcggtgcaaccattaccccgctgaatatggcgtcaacacatatcgttgccgacccaactagaaccagaaaattattactcaataaacgagaactcgattcactctttggtaaagtgaaccgagatggaatgactgttgttgccctttccctttattggaaagccgcttgggcaaaagtgaaaattggtgtggcaaaaggcaaaaaattacacgataaacgtgaagatattaaagaccgcgaatggcaagttgctaaacaacgtattatgaaaaacgcgaaccgtggttaa

SEQ ID NO: 192 - DNA, 477 bp, Haemophilus parasuis
atgagtaaaaaaccaaaagtagcttcaaacacgattgccttaaataaacgtgccagacacgaatattttatcgaagaagaaatcgaagctggtctagaattacaaggctgggaagtcaaatccctgcgagcaggcaaagccaatatcggcgatagctatgtcactttccgtaatggcgaagcctttttattcggtggcactattaccccgttaaatgtcgcttctacccatattgtgtgcgacccaacccgtacccgtaaattattgttaaataagcgtgagttagacacgctttatggtaaagtcagccgtgatgggtttaccgttgtcgccctgtcgctctactggaaaaatgcgtgggcgaaggtcaaaatcggcttggcgaaagggaaaaaattgcacgataaacgtgaagatattaaagaccgtgagtggcaagttgctaaacagcggattatgaagaatgcgaataggtag

SEQ ID NO: 193 - DNA, 477 bp, Haemophilus parasuis
atgagtaaaaaaccaaaagtagcttcaaatacgattgccttaaataaacgtgccagacacgaatattttatcgaagaagaaatcgaagctggtctagaattacaaggctgggaagtcaaatccctgcgagcaggtaaagccaatatcggtgatagttatgtgacatttcgcaacggcgaagcctttttattcggtggcactattaccccgttaaatgtcgcttctacccatattgtgtgcgatccaacccgtacccgtaagttattgttaaataagcgtgagttagacacgctttatggtaaagtcagccgtgatgggtttaccgttgtcgctctgtcgctttactggaaaaatgcgtgggcgaaagtcaaaatcggcttggcgaaagggaaaaaattgcacgataagcgtgaagatattaaagaccgtgagtggcaagttgctaaacagcggattatgaagaatgcgaataggtag